European Patent Specification EP 3 585 159 B1, published May 14, 2025. Title: CAS-READY MOUSE EMBRYONIC STEM CELLS AND MICE AND USES THEREOF. Applicant: Regeneron Pharmaceuticals, Inc. The sequence listing filed with the application follows.

SEQUENCE LISTING (38 sequences)

SEQ ID NO: 1 - DNA, 8628 bp, Artificial Sequence
  Synthetic
  misc_feature (1)..(170): Mouse Rosa26 Upstream
  misc_feature (300)..(333): LoxP
  misc_feature (424)..(2489): Neo-PolyA
  misc_feature (2517)..(2550): LoxP
  misc_feature (2599)..(2608): Kozak
  misc_feature (2605)..(6777): Cas9
  misc_feature (2614)..(2634): Monopartite NLS
  misc_feature (6730)..(6777): Bipartite NLS
  misc_feature (6778)..(6843): P2A
  misc_feature (6844)..(7557): eGFP
  misc_feature (7607)..(8203): WPRE
  misc_feature (8204)..(8419): bGH polyA
  misc_feature (8479)..(8628): Mouse Rosa26 Downstream
ctgcagtggagtaggcggggagaaggccgcacccttctccggaggggggaggggagtgttgcaatacctttctgggagttctctgctgcctcctggcttctgaggaccgccctgggcctgggagaatcccttccccctcttccctcgtgatctgcaactccagtctttctagttgaccagctcggcggtgacctgcacgtctagggcgcagtagtccagggtttccttgatgatgtcatacttatcctgtcccttttttttccacagggcgcgccactagtggatccggaacccttaatataacttcgtataatgtatgctatacgaagttattaggtccctcgacctgcaggaattgttgacaattaatcatcggcatagtatatcggcatagtataatacgacaaggtgaggaactaaaccatgggatcggccattgaacaagatggattgcacgcaggttctccggccgcttgggtggagaggctattcggctatgactgggcacaacagacaatcggctgctctgatgccgccgtgttccggctgtcagcgcaggggcgcccggttctttttgtcaagaccgacctgtccggtgccctgaatgaactgcaggacgaggcagcgcggctatcgtggctggccacgacgggcgttccttgcgcagctgtgctcgacgttgtcactgaagcgggaagggactggctgctattgggcgaagtgccggggcaggatctcctgtcatctcaccttgctcctgccgagaaagtatccatcatggctgatgcaatgcggcggctgcatacgcttgatccggctacctgcccattcgaccaccaagcgaaacatcgcatcgagcgagcacgtactcggatggaagccggtcttgtcgatcaggatgatctggacgaagagcatcaggggctcgcgccagccgaactgttcgccaggctcaaggcgcgcatgcccgacggcgatgatctcgtcgtgacccatggcgatgcctgcttgccgaatatcatggtggaaaatggccgcttttctggattcatcgactgtggccggctgggtgtggcggaccgctatcaggacatagcgttggctacccgtgatattgctgaagagcttggcggcgaatgggctgaccgcttcctcgtgctttacggtatcgccgctcccgattcgcagcgcatcgccttctatcgccttcttgacgagttcttctgaggggatccgctgtaagtctgcagaaattgatgatctattaaacaataaagatgtccactaaaatggaagtttttcctgtcatactttgttaagaagggtgagaacagagtacctacattttgaatggaaggattggagctacgggggtgggggtggggtgggattagataaatgcctgctctttactgaaggctctttactattgctttatgataatgtttcatagttggatatcataatttaaacaagcaaaaccaaattaagggccagctcattcctcccactcatgatctatagatctatagatctctcgtgggatcattgtttttctcttgattcccactttgtggttctaagtactgtggtttccaaatgtgtcagtttcatagcctgaagaacgagatcagcagcctctgttccacatacacttcattctcagtattgttttgccaagttctaattccatcagaagcttgcagatctgcgactctagaggatctgcgactctagaggatcataatcagccataccacatttgtagaggttttacttgctttaaaaaacctcccacacctccccctgaacctgaaacataaaatgaatgcaattgttgttgttaacttgtttattgcagcttataatggttacaaataaagcaatagcatcacaaatttcacaaataaagcatttttttcactgcattctagttgtggtttgtccaaactcatcaatgtatcttatcatgtctggatctgcgactctagaggatcataatcagccataccacatttgtagaggttttacttgctttaaaaaacctcccacacctccccctgaacctgaaacataaaatgaatgcaattgttgttgttaacttgtttattgcagcttataatggttacaaataaagcaatagcatcacaaatttcacaaataaagcatttttttcactgcattctagttgtggtttgtccaaactcatcaatgtatcttatcatgtctggatctgcgactctagaggatcataatcagccataccacatttgtagaggttttacttgctttaaaaaacctcccacacctccccctgaacctgaaacataaaatgaatgcaattgttgttgttaacttgtttattgcagcttataatggttacaaataaagcaatagcatcacaaatttcacaaataaagcatttttttcactgcattctagttgtggtttgtccaaactcatcaatgtatcttatcatgtctggatccccatcaagctgatccggaacccttaatataacttcgtataatgtatgctatacgaagttattaggtccctcgacctgcagcccaagctagtgcccgggaattcgctagggccaccatggacaagcccaagaaaaagcggaaagtgaagtacagcatcggcctggacatcggcaccaactctgtgggctgggccgtgatcaccgacgagtacaaggtgcccagcaagaaattcaaggtgctgggcaacaccgacaggcacagcatcaagaagaacctgatcggcgccctgctgttcgacagcggcgaaacagccgaggccaccagactgaagagaaccgccagaagaagatacaccaggcggaagaacaggatctgctatctgcaagagatcttcagcaacgagatggccaaggtggacgacagcttcttccacagactggaagagtccttcctggtggaagaggacaagaagcacgagagacaccccatcttcggcaacatcgtggacgaggtggcctaccacgagaagtaccccaccatctaccacctgagaaagaaactggtggacagcaccgacaaggccgacctgagactgatctacctggccctggcccacatgatcaagttcagaggccacttcctgatcgagggcgacctgaaccccgacaacagcgacgtggacaagctgttcatccagctggtgcagacctacaaccagctgttcgaggaaaaccccatcaacgccagcggcgtggacgccaaggctatcctgtctgccagactgagcaagagcagaaggctggaaaatctgatcgcccagctgcccggcgagaagaagaacggcctgttcggcaacctgattgccctgagcctgggcctgacccccaacttcaagagcaacttcgacctggccgaggatgccaaactgcagctgagcaaggacacctacgacgacgacctggacaacctgctggcccagatcggcgaccagtacgccgacctgttcctggccgccaagaacctgtctgacgccatcctgctgagcgacatcctgagagtgaacaccgagatcaccaaggcccccctgagcgcctctatgatcaagagatacgacgagcaccaccaggacctgaccctgctgaaagctctcgtgcggcagcagctgcctgagaagtacaaagaaatcttcttcgaccagagcaagaacggctacgccggctacatcgatggcggcgctagccaggaagagttctacaagttcatcaagcccatcctggaaaagatggacggcaccgaggaactgctcgtgaagctgaacagagaggacctgctgagaaagcagagaaccttcgacaacggcagcatcccccaccagatccacctgggagagctgcacgctatcctgagaaggcaggaagatttttacccattcctgaaggacaaccgggaaaagatcgagaagatcctgaccttcaggatcccctactacgtgggccccctggccagaggcaacagcagattcgcctggatgaccagaaagagcgaggaaaccatcaccccctggaacttcgaggaagtggtggacaagggcgccagcgcccagagcttcatcgagagaatgacaaacttcgataagaacctgcccaacgagaaggtgctgcccaagcacagcctgctgtacgagtacttcaccgtgtacaacgagctgaccaaagtgaaatacgtgaccgagggaatgagaaagcccgccttcctgagcggcgagcagaaaaaggccatcgtggacctgctgttcaagaccaacagaaaagtgaccgtgaagcagctgaaagaggactacttcaagaaaatcgagtgcttcgactccgtggaaatctccggcgtggaagatagattcaacgcctccctgggcacataccacgatctgctgaaaattatcaaggacaaggacttcctggataacgaagagaacgaggacattctggaagatatcgtgctgaccctgacactgtttgaggaccgcgagatgatcgaggaaaggctgaaaacctacgctcacctgttcgacgacaaagtgatgaagcagctgaagagaaggcggtacaccggctggggcaggctgagcagaaagctgatcaacggcatcagagacaagcagagcggcaagacaatcctggatttcctgaagtccgacggcttcgccaaccggaacttcatgcagctgatccacgacgacagcctgacattcaaagaggacatccagaaagcccaggtgtccggccagggcgactctctgcacgagcatatcgctaacctggccggcagccccgctatcaagaagggcatcctgcagacagtgaaggtggtggacgagctcgtgaaagtgatgggcagacacaagcccgagaacatcgtgatcgagatggctagagagaaccagaccacccagaagggacagaagaactcccgcgagaggatgaagagaatcgaagagggcatcaaagagctgggcagccagatcctgaaagaacaccccgtggaaaacacccagctgcagaacgagaagctgtacctgtactacctgcagaatggccgggatatgtacgtggaccaggaactggacatcaacagactgtccgactacgatgtggaccatatcgtgcctcagagctttctgaaggacgactccatcgataacaaagtgctgactcggagcgacaagaacagaggcaagagcgacaacgtgccctccgaagaggtcgtgaagaagatgaagaactactggcgacagctgctgaacgccaagctgattacccagaggaagttcgataacctgaccaaggccgagagaggcggcctgagcgagctggataaggccggcttcatcaagaggcagctggtggaaaccagacagatcacaaagcacgtggcacagatcctggactcccggatgaacactaagtacgacgaaaacgataagctgatccgggaagtgaaagtgatcaccctgaagtccaagctggtgtccgatttccggaaggatttccagttttacaaagtgcgcgagatcaacaactaccaccacgcccacgacgcctacctgaacgccgtcgtgggaaccgccctgatcaaaaagtaccctaagctggaaagcgagttcgtgtacggcgactacaaggtgtacgacgtgcggaagatgatcgccaagagcgagcaggaaatcggcaaggctaccgccaagtacttcttctacagcaacatcatgaactttttcaagaccgaaatcaccctggccaacggcgagatcagaaagcgccctctgatcgagacaaacggcgaaaccggggagatcgtgtgggataagggcagagacttcgccacagtgcgaaaggtgctgagcatgccccaagtgaatatcgtgaaaaagaccgaggtgcagacaggcggcttcagcaaagagtctatcctgcccaagaggaacagcgacaagctgatcgccagaaagaaggactgggaccccaagaagtacggcggcttcgacagccctaccgtggcctactctgtgctggtggtggctaaggtggaaaagggcaagtccaagaaactgaagagtgtgaaagagctgctggggatcaccatcatggaaagaagcagctttgagaagaaccctatcgactttctggaagccaagggctacaaagaagtgaaaaaggacctgatcatcaagctgcctaagtactccctgttcgagctggaaaacggcagaaagagaatgctggcctctgccggcgaactgcagaagggaaacgagctggccctgcctagcaaatatgtgaacttcctgtacctggcctcccactatgagaagctgaagggcagccctgaggacaacgaacagaaacagctgtttgtggaacagcataagcactacctggacgagatcatcgagcagatcagcgagttctccaagagagtgatcctggccgacgccaatctggacaaggtgctgtctgcctacaacaagcacagggacaagcctatcagagagcaggccgagaatatcatccacctgttcaccctgacaaacctgggcgctcctgccgccttcaagtactttgacaccaccatcgaccggaagaggtacaccagcaccaaagaggtgctggacgccaccctgatccaccagagcatcaccggcctgtacgagacaagaatcgacctgtctcagctgggaggcgacaagagacctgccgccactaagaaggccggacaggccaaaaagaagaagggaagcggagccactaacttctccctgttgaaacaagcaggggatgtcgaagagaatcccgggccagtgagcaagggcgaggagctgttcaccggggtggtgcccatcctggtcgagctggacggcgacgtaaacggccacaagttcagcgtgtccggcgagggcgagggcgatgccacctacggcaagctgaccctgaagttcatctgcaccaccggcaagctgcccgtgccctggcccaccctcgtgaccaccctgacctacggcgtgcagtgcttcagccgctaccccgaccacatgaagcagcacgacttcttcaagtccgccatgcccgaaggctacgtccaggagcgcaccatcttcttcaaggacgacggcaactacaagacccgcgccgaggtgaagttcgagggcgacaccctggtgaaccgcatcgagctgaagggcatcgacttcaaggaggacggcaacatcctggggcacaagctggagtacaactacaacagccacaacgtctatatcatggccgacaagcagaagaacggcatcaaggtgaacttcaagatccgccacaacatcgaggacggcagcgtgcagctcgccgaccactaccagcagaacacccccatcggcgacggccccgtgctgctgcccgacaaccactacctgagcacccagtccgccctgagcaaagaccccaacgagaagcgcgatcacatggtcctgctggagttcgtgaccgccgccgggatcactctcggcatggacgagctgtacaagtaaacgcgtatgcatggccggccctgcaggaattcgatatcaagcttatcgataatcaacctctggattacaaaatttgtgaaagattgactggtattcttaactatgttgctccttttacgctatgtggatacgctgctttaatgcctttgtatcatgctattgcttcccgtatggctttcattttctcctccttgtataaatcctggttgctgtctctttatgaggagttgtggcccgttgtcaggcaacgtggcgtggtgtgcactgtgtttgctgacgcaacccccactggttggggcattgccaccacctgtcagctcctttccgggactttcgctttccccctccctattgccacggcggaactcatcgccgcctgccttgcccgctgctggacaggggctcggctgttgggcactgacaattccgtggtgttgtcggggaaatcatcgtcctttccttggctgctcgcctgtgttgccacctggattctgcgcgggacgtccttctgctacgtcccttcggccctcaatccagcggaccttccttcccgcggcctgctgccggctctgcggcctcttccgcgtcttcgccttcgccctcagacgagtcggatctccctttgggccgcctccccgcatcgcgacctcgacctcgactgtgccttctagttgccagccatctgttgtttgcccctcccccgtgccttccttgaccctggaaggtgccactcccactgtcctttcctaataaaatgaggaaattgcatcgcattgtctgagtaggtgtcattctattctggggggtggggtggggcaggacagcaagggggaggattgggaagacaatggcaggcatgctggggaactagtggtgccagggcgtgcccttgggctccccgggcgcggcggccatcgctcgagtaaaattggagggacaagacttcccacagattttcggttttgtcgggaagttttttaataggggcaaataaggaaaatgggaggataggtagtcatctggggttttatgcagcaaaactacaggttattattgcttgtgatccgc

SEQ ID NO: 2 - protein, 18 aa, Artificial Sequence
  Synthetic
EGRGSLLTCGDVEENPGP

SEQ ID NO: 3 - protein, 19 aa, Artificial Sequence
  Synthetic
ATNFSLLKQAGDVEENPGP

SEQ ID NO: 4 - protein, 20 aa, Artificial Sequence
  Synthetic
QCTNYALLKLAGDVESNPGP

SEQ ID NO: 5 - protein, 22 aa, Artificial Sequence
  Synthetic
VKQTLNFDLLKLAGDVESNPGP

SEQ ID NO: 6 - RNA, 82 nt, Artificial Sequence
  Synthetic
guuggaaccauucaaaacagcauagcaaguuaaaauaaggcuaguccguuaucaacuugaaaaaguggcaccgagucggugc

SEQ ID NO: 7 - RNA, 76 nt, Artificial Sequence
  Synthetic
guuuuagagcuagaaauagcaaguuaaaauaaggcuaguccguuaucaacuugaaaaaguggcaccgagucggugc

SEQ ID NO: 8 - RNA, 86 nt, Artificial Sequence
  Synthetic
guuuaagagcuaugcuggaaacagcauagcaaguuuaaauaaggcuaguccguuaucaacuugaaaaaguggcaccgagucggugc

SEQ ID NO: 9 - DNA, 23 bp, Artificial Sequence
  Synthetic
  misc_feature (2)..(21): n = A, T, C, or G
gnnnnnnnnnnnnnnnnnnnngg

SEQ ID NO: 10 - DNA, 23 bp, Artificial Sequence
  Synthetic
  misc_feature (1)..(21): n = A, T, C, or G
nnnnnnnnnnnnnnnnnnnnngg

SEQ ID NO: 11 - DNA, 25 bp, Artificial Sequence
  Synthetic
  misc_feature (3)..(23): n = A, T, C, or G
ggnnnnnnnnnnnnnnnnnnnnngg

SEQ ID NO: 12 - DNA, 6411 bp, Artificial Sequence
  Synthetic
  misc_feature (1)..(170): Mouse Rosa26 Upstream
  misc_feature (300)..(333): LoxP
  misc_feature (382)..(391): Kozak
  misc_feature (388)..(4560): Cas9
  misc_feature (397)..(417): Monopartite NLS
  misc_feature (4513)..(4560): Bipartite NLS
  misc_feature (4561)..(4626): P2A
  misc_feature (4627)..(5340): eGFP
  misc_feature (5390)..(5986): WPRE
  misc_feature (5987)..(6202): bGH PolyA
  misc_feature (6262)..(6411): Mouse Rosa26 Downstream
ctgcagtggagtaggcggggagaaggccgcacccttctccggaggggggaggggagtgttgcaatacctttctgggagttctctgctgcctcctggcttctgaggaccgccctgggcctgggagaatcccttccccctcttccctcgtgatctgcaactccagtctttctagttgaccagctcggcggtgacctgcacgtctagggcgcagtagtccagggtttccttgatgatgtcatacttatcctgtcccttttttttccacagggcgcgccactagtggatccggaacccttaatataacttcgtataatgtatgctatacgaagttattaggtccctcgacctgcagcccaagctagtgcccgggaattcgctagggccaccatggacaagcccaagaaaaagcggaaagtgaagtacagcatcggcctggacatcggcaccaactctgtgggctgggccgtgatcaccgacgagtacaaggtgcccagcaagaaattcaaggtgctgggcaacaccgacaggcacagcatcaagaagaacctgatcggcgccctgctgttcgacagcggcgaaacagccgaggccaccagactgaagagaaccgccagaagaagatacaccaggcggaagaacaggatctgctatctgcaagagatcttcagcaacgagatggccaaggtggacgacagcttcttccacagactggaagagtccttcctggtggaagaggacaagaagcacgagagacaccccatcttcggcaacatcgtggacgaggtggcctaccacgagaagtaccccaccatctaccacctgagaaagaaactggtggacagcaccgacaaggccgacctgagactgatctacctggccctggcccacatgatcaagttcagaggccacttcctgatcgagggcgacctgaaccccgacaacagcgacgtggacaagctgttcatccagctggtgcagacctacaaccagctgttcgaggaaaaccccatcaacgccagcggcgtggacgccaaggctatcctgtctgccagactgagcaagagcagaaggctggaaaatctgatcgcccagctgcccggcgagaagaagaacggcctgttcggcaacctgattgccctgagcctgggcctgacccccaacttcaagagcaacttcgacctggccgaggatgccaaactgcagctgagcaaggacacctacgacgacgacctggacaacctgctggcccagatcggcgaccagtacgccgacctgttcctggccgccaagaacctgtctgacgccatcctgctgagcgacatcctgagagtgaacaccgagatcaccaaggcccccctgagcgcctctatgatcaagagatacgacgagcaccaccaggacctgaccctgctgaaagctctcgtgcggcagcagctgcctgagaagtacaaagaaatcttcttcgaccagagcaagaacggctacgccggctacatcgatggcggcgctagccaggaagagttctacaagttcatcaagcccatcctggaaaagatggacggcaccgaggaactgctcgtgaagctgaacagagaggacctgctgagaaagcagagaaccttcgacaacggcagcatcccccaccagatccacctgggagagctgcacgctatcctgagaaggcaggaagatttttacccattcctgaaggacaaccgggaaaagatcgagaagatcctgaccttcaggatcccctactacgtgggccccctggccagaggcaacagcagattcgcctggatgaccagaaagagcgaggaaaccatcaccccctggaacttcgaggaagtggtggacaagggcgccagcgcccagagcttcatcgagagaatgacaaacttcgataagaacctgcccaacgagaaggtgctgcccaagcacagcctgctgtacgagtacttcaccgtgtacaacgagctgaccaaagtgaaatacgtgaccgagggaatgagaaagcccgccttcctgagcggcgagcagaaaaaggccatcgtggacctgctgttcaagaccaacagaaaagtgaccgtgaagcagctgaaagaggactacttcaagaaaatcgagtgcttcgactccgtggaaatctccggcgtggaagatagattcaacgcctccctgggcacataccacgatctgctgaaaattatcaaggacaaggacttcctggataacgaagagaacgaggacattctggaagatatcgtgctgaccctgacactgtttgaggaccgcgagatgatcgaggaaaggctgaaaacctacgctcacctgttcgacgacaaagtgatgaagcagctgaagagaaggcggtacaccggctggggcaggctgagcagaaagctgatcaacggcatcagagacaagcagagcggcaagacaatcctggatttcctgaagtccgacggcttcgccaaccggaacttcatgcagctgatccacgacgacagcctgacattcaaagaggacatccagaaagcccaggtgtccggccagggcgactctctgcacgagcatatcgctaacctggccggcagccccgctatcaagaagggcatcctgcagacagtgaaggtggtggacgagctcgtgaaagtgatgggcagacacaagcccgagaacatcgtgatcgagatggctagagagaaccagaccacccagaagggacagaagaactcccgcgagaggatgaagagaatcgaagagggcatcaaagagctgggcagccagatcctgaaagaacaccccgtggaaaacacccagctgcagaacgagaagctgtacctgtactacctgcagaatggccgggatatgtacgtggaccaggaactggacatcaacagactgtccgactacgatgtggaccatatcgtgcctcagagctttctgaaggacgactccatcgataacaaagtgctgactcggagcgacaagaacagaggcaagagcgacaacgtgccctccgaagaggtcgtgaagaagatgaagaactactggcgacagctgctgaacgccaagctgattacccagaggaagttcgataacctgaccaaggccgagagaggcggcctgagcgagctggataaggccggcttcatcaagaggcagctggtggaaaccagacagatcacaaagcacgtggcacagatcctggactcccggatgaacactaagtacgacgaaaacgataagctgatccgggaagtgaaagtgatcaccctgaagtccaagctggtgtccgatttccggaaggatttccagttttacaaagtgcgcgagatcaacaactaccaccacgcccacgacgcctacctgaacgccgtcgtgggaaccgccctgatcaaaaagtaccctaagctggaaagcgagttcgtgtacggcgactacaaggtgtacgacgtgcggaagatgatcgccaagagcgagcaggaaatcggcaaggctaccgccaagtacttcttctacagcaacatcatgaactttttcaagaccgaaatcaccctggccaacggcgagatcagaaagcgccctctgatcgagacaaacggcgaaaccggggagatcgtgtgggataagggcagagacttcgccacagtgcgaaaggtgctgagcatgccccaagtgaatatcgtgaaaaagaccgaggtgcagacaggcggcttcagcaaagagtctatcctgcccaagaggaacagcgacaagctgatcgccagaaagaaggactgggaccccaagaagtacggcggcttcgacagccctaccgtggcctactctgtgctggtggtggctaaggtggaaaagggcaagtccaagaaactgaagagtgtgaaagagctgctggggatcaccatcatggaaagaagcagctttgagaagaaccctatcgactttctggaagccaagggctacaaagaagtgaaaaaggacctgatcatcaagctgcctaagtactccctgttcgagctggaaaacggcagaaagagaatgctggcctctgccggcgaactgcagaagggaaacgagctggccctgcctagcaaatatgtgaacttcctgtacctggcctcccactatgagaagctgaagggcagccctgaggacaacgaacagaaacagctgtttgtggaacagcataagcactacctggacgagatcatcgagcagatcagcgagttctccaagagagtgatcctggccgacgccaatctggacaaggtgctgtctgcctacaacaagcacagggacaagcctatcagagagcaggccgagaatatcatccacctgttcaccctgacaaacctgggcgctcctgccgccttcaagtactttgacaccaccatcgaccggaagaggtacaccagcaccaaagaggtgctggacgccaccctgatccaccagagcatcaccggcctgtacgagacaagaatcgacctgtctcagctgggaggcgacaagagacctgccgccactaagaaggccggacaggccaaaaagaagaagggaagcggagccactaacttctccctgttgaaacaagcaggggatgtcgaagagaatcccgggccagtgagcaagggcgaggagctgttcaccggggtggtgcccatcctggtcgagctggacggcgacgtaaacggccacaagttcagcgtgtccggcgagggcgagggcgatgccacctacggcaagctgaccctgaagttcatctgcaccaccggcaagctgcccgtgccctggcccaccctcgtgaccaccctgacctacggcgtgcagtgcttcagccgctaccccgaccacatgaagcagcacgacttcttcaagtccgccatgcccgaaggctacgtccaggagcgcaccatcttcttcaaggacgacggcaactacaagacccgcgccgaggtgaagttcgagggcgacaccctggtgaaccgcatcgagctgaagggcatcgacttcaaggaggacggcaacatcctggggcacaagctggagtacaactacaacagccacaacgtctatatcatggccgacaagcagaagaacggcatcaaggtgaacttcaagatccgccacaacatcgaggacggcagcgtgcagctcgccgaccactaccagcagaacacccccatcggcgacggccccgtgctgctgcccgacaaccactacctgagcacccagtccgccctgagcaaagaccccaacgagaagcgcgatcacatggtcctgctggagttcgtgaccgccgccgggatcactctcggcatggacgagctgtacaagtaaacgcgtatgcatggccggccctgcaggaattcgatatcaagcttatcgataatcaacctctggattacaaaatttgtgaaagattgactggtattcttaactatgttgctccttttacgctatgtggatacgctgctttaatgcctttgtatcatgctattgcttcccgtatggctttcattttctcctccttgtataaatcctggttgctgtctctttatgaggagttgtggcccgttgtcaggcaacgtggcgtggtgtgcactgtgtttgctgacgcaacccccactggttggggcattgccaccacctgtcagctcctttccgggactttcgctttccccctccctattgccacggcggaactcatcgccgcctgccttgcccgctgctggacaggggctcggctgttgggcactgacaattccgtggtgttgtcggggaaatcatcgtcctttccttggctgctcgcctgtgttgccacctggattctgcgcgggacgtccttctgctacgtcccttcggccctcaatccagcggaccttccttcccgcggcctgctgccggctctgcggcctcttccgcgtcttcgccttcgccctcagacgagtcggatctccctttgggccgcctccccgcatcgcgacctcgacctcgactgtgccttctagttgccagccatctgttgtttgcccctcccccgtgccttccttgaccctggaaggtgccactcccactgtcctttcctaataaaatgaggaaattgcatcgcattgtctgagtaggtgtcattctattctggggggtggggtggggcaggacagcaagggggaggattgggaagacaatggcaggcatgctggggaactagtggtgccagggcgtgcccttgggctccccgggcgcggcggccatcgctcgagtaaaattggagggacaagacttcccacagattttcggttttgtcgggaagttttttaataggggcaaataaggaaaatgggaggataggtagtcatctggggttttatgcagcaaaactacaggttattattgcttgtgatccgc

SEQ ID NO: 13 - protein, 1651 aa, Artificial Sequence
  Synthetic
  MISC_FEATURE (1)..(1391): Cas9
  MISC_FEATURE (1392)..(1413): P2A
  MISC_FEATURE (1414)..(1651): eGFP
MDKPKKKRKVKYSIGLDIGTNSVGWAVITDEYKVPSKKFKVLGNTDRHSIKKNLIGALLFDSGETAEATRLKRTARRRYTRRKNRICYLQEIFSNEMAKVDDSFFHRLEESFLVEEDKKHERHPIFGNIVDEVAYHEKYPTIYHLRKKLVDSTDKADLRLIYLALAHMIKFRGHFLIEGDLNPDNSDVDKLFIQLVQTYNQLFEENPINASGVDAKAILSARLSKSRRLENLIAQLPGEKKNGLFGNLIALSLGLTPNFKSNFDLAEDAKLQLSKDTYDDDLDNLLAQIGDQYADLFLAAKNLSDAILLSDILRVNTEITKAPLSASMIKRYDEHHQDLTLLKALVRQQLPEKYKEIFFDQSKNGYAGYIDGGASQEEFYKFIKPILEKMDGTEELLVKLNREDLLRKQRTFDNGSIPHQIHLGELHAILRRQEDFYPFLKDNREKIEKILTFRIPYYVGPLARGNSRFAWMTRKSEETITPWNFEEVVDKGASAQSFIERMTNFDKNLPNEKVLPKHSLLYEYFTVYNELTKVKYVTEGMRKPAFLSGEQKKAIVDLLFKTNRKVTVKQLKEDYFKKIECFDSVEISGVEDRFNASLGTYHDLLKIIKDKDFLDNEENEDILEDIVLTLTLFEDREMIEERLKTYAHLFDDKVMKQLKRRRYTGWGRLSRKLINGIRDKQSGKTILDFLKSDGFANRNFMQLIHDDSLTFKEDIQKAQVSGQGDSLHEHIANLAGSPAIKKGILQTVKVVDELVKVMGRHKPENIVIEMARENQTTQKGQKNSRERMKRIEEGIKELGSQILKEHPVENTQLQNEKLYLYYLQNGRDMYVDQELDINRLSDYDVDHIVPQSFLKDDSIDNKVLTRSDKNRGKSDNVPSEEVVKKMKNYWRQLLNAKLITQRKFDNLTKAERGGLSELDKAGFIKRQLVETRQITKHVAQILDSRMNTKYDENDKLIREVKVITLKSKLVSDFRKDFQFYKVREINNYHHAHDAYLNAVVGTALIKKYPKLESEFVYGDYKVYDVRKMIAKSEQEIGKATAKYFFYSNIMNFFKTEITLANGEIRKRPLIETNGETGEIVWDKGRDFATVRKVLSMPQVNIVKKTEVQTGGFSKESILPKRNSDKLIARKKDWDPKKYGGFDSPTVAYSVLVVAKVEKGKSKKLKSVKELLGITIMERSSFEKNPIDFLEAKGYKEVKKDLIIKLPKYSLFELENGRKRMLASAGELQKGNELALPSKYVNFLYLASHYEKLKGSPEDNEQKQLFVEQHKHYLDEIIEQISEFSKRVILADANLDKVLSAYNKHRDKPIREQAENIIHLFTLTNLGAPAAFKYFDTTIDRKRYTSTKEVLDATLIHQSITGLYETRIDLSQLGGDKRPAATKKAGQAKKKKGSGATNFSLLKQAGDVEENPGPVSKGEELFTGVVPILVELDGDVNGHKFSVSGEGEGDATYGKLTLKFICTTGKLPVPWPTLVTTLTYGVQCFSRYPDHMKQHDFFKSAMPEGYVQERTIFFKDDGNYKTRAEVKFEGDTLVNRIELKGIDFKEDGNILGHKLEYNYNSHNVYIMADKQKNGIKVNFKIRHNIEDGSVQLADHYQQNTPIGDGPVLLPDNHYLSTQSALSKDPNEKRDHMVLLEFVTAAGITLGMDELYK

SEQ ID NO: 14 - DNA, 10439 bp, Artificial Sequence
  Synthetic
  misc_feature (1)..(170): Mouse Rosa26 Upstream
  misc_feature (195)..(1913): CAGG Promoter
  misc_feature (1996)..(2029): LoxP
  misc_feature (2120)..(4185): Neo-PolyA
  misc_feature (4213)..(4246): LoxP
  misc_feature (4341)..(4350): Kozak
  misc_feature (4350)..(4415): 3xFLAG
  misc_feature (4416)..(8588): Cas9
  misc_feature (4425)..(4445): Monopartite NLS
  misc_feature (8541)..(8588): Bipartite NLS
  misc_feature (8589)..(8654): P2A
  misc_feature (8655)..(9368): eGFP
  misc_feature (9418)..(10014): WPRE
  misc_feature (10015)..(10230): bGH PolyA
  misc_feature (10290)..(10439): Mouse Rosa26 Downstream
ctgcagtggagtaggcggggagaaggccgcacccttctccggaggggggaggggagtgttgcaatacctttctgggagttctctgctgcctcctggcttctgaggaccgccctgggcctgggagaatcccttccccctcttccctcgtgatctgcaactccagtctttctccttaattaaggcctccaaggcctactagttattaatagtaatcaattacggggtcattagttcatagcccatatatggagttccgcgttacataacttacggtaaatggcccgcctggctgaccgcccaacgacccccgcccattgacgtcaataatgacgtatgttcccatagtaacgccaatagggactttccattgacgtcaatgggtggagtatttacggtaaactgcccacttggcagtacatcaagtgtatcatatgccaagtacgccccctattgacgtcaatgacggtaaatggcccgcctggcattatgcccagtacatgaccttatgggactttcctacttggcagtacatctacgtattagtcatcgctattaccatggtcgaggtgagccccacgttctgcttcactctccccatctcccccccctccccacccccaattttgtatttatttattttttaattattttgtgcagcgatgggggcggggggggggggggggcgcgcgccaggcggggcggggcggggcgaggggcggggcggggcgaggcggagaggtgcggcggcagccaatcagagcggcgcgctccgaaagtttccttttatggcgaggcggcggcggcggcggccctataaaaagcgaagcgcgcggcgggcggggagtcgctgcgacgctgccttcgccccgtgccccgctccgccgccgcctcgcgccgcccgccccggctctgactgaccgcgttactcccacaggtgagcgggcgggacggcccttctcctccgggctgtaattagcgcttggtttaatgacggcttgtttcttttctgtggctgcgtgaaagccttgaggggctccgggagggccctttgtgcggggggagcggctcggggggtgcgtgcgtgtgtgtgtgcgtggggagcgccgcgtgcggctccgcgctgcccggcggctgtgagcgctgcgggcgcggcgcggggctttgtgcgctccgcagtgtgcgcgaggggagcgcggccgggggcggtgccccgcggtgcggggggggctgcgaggggaacaaaggctgcgtgcggggtgtgtgcgtgggggggtgagcagggggtgtgggcgcgtcggtcgggctgcaaccccccctgcacccccctccccgagttgctgagcacggcccggcttcgggtgcggggctccgtacggggcgtggcgcggggctcgccgtgccgggcggggggtggcggcaggtgggggtgccgggcggggcggggccgcctcgggccggggagggctcgggggaggggcgcggcggcccccggagcgccggcggctgtcgaggcgcggcgagccgcagccattgccttttatggtaatcgtgcgagagggcgcagggacttcctttgtcccaaatctgtgcggagccgaaatctgggaggcgccgccgcaccccctctagcgggcgcggggcgaagcggtgcggcgccggcaggaaggaaatgggcggggagggccttcgtgcgtcgccgcgccgccgtccccttctccctctccagcctcggggctgtccgcggggggacggctgccttcgggggggacggggcagggcggggttcggcttctggcgtgtgaccggcggctctagagcctctgctaaccatgttcatgccttcttctttttcctacagctcctgggcaacgtgctggttattgtgctgtctcatcattttggcaaagaattcgctaggagaattgatttgataccgcgggccctaagtcgacatttaaatcatttaaatccactagtggatccggaacccttaatataacttcgtataatgtatgctatacgaagttattaggtccctcgacctgcaggaattgttgacaattaatcatcggcatagtatatcggcatagtataatacgacaaggtgaggaactaaaccatgggatcggccattgaacaagatggattgcacgcaggttctccggccgcttgggtggagaggctattcggctatgactgggcacaacagacaatcggctgctctgatgccgccgtgttccggctgtcagcgcaggggcgcccggttctttttgtcaagaccgacctgtccggtgccctgaatgaactgcaggacgaggcagcgcggctatcgtggctggccacgacgggcgttccttgcgcagctgtgctcgacgttgtcactgaagcgggaagggactggctgctattgggcgaagtgccggggcaggatctcctgtcatctcaccttgctcctgccgagaaagtatccatcatggctgatgcaatgcggcggctgcatacgcttgatccggctacctgcccattcgaccaccaagcgaaacatcgcatcgagcgagcacgtactcggatggaagccggtcttgtcgatcaggatgatctggacgaagagcatcaggggctcgcgccagccgaactgttcgccaggctcaaggcgcgcatgcccgacggcgatgatctcgtcgtgacccatggcgatgcctgcttgccgaatatcatggtggaaaatggccgcttttctggattcatcgactgtggccggctgggtgtggcggaccgctatcaggacatagcgttggctacccgtgatattgctgaagagcttggcggcgaatgggctgaccgcttcctcgtgctttacggtatcgccgctcccgattcgcagcgcatcgccttctatcgccttcttgacgagttcttctgaggggatccgctgtaagtctgcagaaattgatgatctattaaacaataaagatgtccactaaaatggaagtttttcctgtcatactttgttaagaagggtgagaacagagtacctacattttgaatggaaggattggagctacgggggtgggggtggggtgggattagataaatgcctgctctttactgaaggctctttactattgctttatgataatgtttcatagttggatatcataatttaaacaagcaaaaccaaattaagggccagctcattcctcccactcatgatctatagatctatagatctctcgtgggatcattgtttttctcttgattcccactttgtggttctaagtactgtggtttccaaatgtgtcagtttcatagcctgaagaacgagatcagcagcctctgttccacatacacttcattctcagtattgttttgccaagttctaattccatcagaagcttgcagatctgcgactctagaggatctgcgactctagaggatcataatcagccataccacatttgtagaggttttacttgctttaaaaaacctcccacacctccccctgaacctgaaacataaaatgaatgcaattgttgttgttaacttgtttattgcagcttataatggttacaaataaagcaatagcatcacaaatttcacaaataaagcatttttttcactgcattctagttgtggtttgtccaaactcatcaatgtatcttatcatgtctggatctgcgactctagaggatcataatcagccataccacatttgtagaggttttacttgctttaaaaaacctcccacacctccccctgaacctgaaacataaaatgaatgcaattgttgttgttaacttgtttattgcagcttataatggttacaaataaagcaatagcatcacaaatttcacaaataaagcatttttttcactgcattctagttgtggtttgtccaaactcatcaatgtatcttatcatgtctggatctgcgactctagaggatcataatcagccataccacatttgtagaggttttacttgctttaaaaaacctcccacacctccccctgaacctgaaacataaaatgaatgcaattgttgttgttaacttgtttattgcagcttataatggttacaaataaagcaatagcatcacaaatttcacaaataaagcatttttttcactgcattctagttgtggtttgtccaaactcatcaatgtatcttatcatgtctggatccccatcaagctgatccggaacccttaatataacttcgtataatgtatgctatacgaagttattaggtccctcgacctgcagcccaagctagtgcccgggtaggtccctcgacctgcagcccaagctagatcgaattcggccggccttcgaacacgtgccaccatggactataaggaccacgacggagactacaaggatcatgatattgattacaaagacgatgacgataagatggacaagcccaagaaaaagcggaaagtgaagtacagcatcggcctggacatcggcaccaactctgtgggctgggccgtgatcaccgacgagtacaaggtgcccagcaagaaattcaaggtgctgggcaacaccgacaggcacagcatcaagaagaacctgatcggcgccctgctgttcgacagcggcgaaacagccgaggccaccagactgaagagaaccgccagaagaagatacaccaggcggaagaacaggatctgctatctgcaagagatcttcagcaacgagatggccaaggtggacgacagcttcttccacagactggaagagtccttcctggtggaagaggacaagaagcacgagagacaccccatcttcggcaacatcgtggacgaggtggcctaccacgagaagtaccccaccatctaccacctgagaaagaaactggtggacagcaccgacaaggccgacctgagactgatctacctggccctggcccacatgatcaagttcagaggccacttcctgatcgagggcgacctgaaccccgacaacagcgacgtggacaagctgttcatccagctggtgcagacctacaaccagctgttcgaggaaaaccccatcaacgccagcggcgtggacgccaaggctatcctgtctgccagactgagcaagagcagaaggctggaaaatctgatcgcccagctgcccggcgagaagaagaacggcctgttcggcaacctgattgccctgagcctgggcctgacccccaacttcaagagcaacttcgacctggccgaggatgccaaactgcagctgagcaaggacacctacgacgacgacctggacaacctgctggcccagatcggcgaccagtacgccgacctgttcctggccgccaagaacctgtctgacgccatcctgctgagcgacatcctgagagtgaacaccgagatcaccaaggcccccctgagcgcctctatgatcaagagatacgacgagcaccaccaggacctgaccctgctgaaagctctcgtgcggcagcagctgcctgagaagtacaaagaaatcttcttcgaccagagcaagaacggctacgccggctacatcgatggcggcgctagccaggaagagttctacaagttcatcaagcccatcctggaaaagatggacggcaccgaggaactgctcgtgaagctgaacagagaggacctgctgagaaagcagagaaccttcgacaacggcagcatcccccaccagatccacctgggagagctgcacgctatcctgagaaggcaggaagatttttacccattcctgaaggacaaccgggaaaagatcgagaagatcctgaccttcaggatcccctactacgtgggccccctggccagaggcaacagcagattcgcctggatgaccagaaagagcgaggaaaccatcaccccctggaacttcgaggaagtggtggacaagggcgccagcgcccagagcttcatcgagagaatgacaaacttcgataagaacctgcccaacgagaaggtgctgcccaagcacagcctgctgtacgagtacttcaccgtgtacaacgagctgaccaaagtgaaatacgtgaccgagggaatgagaaagcccgccttcctgagcggcgagcagaaaaaggccatcgtggacctgctgttcaagaccaacagaaaagtgaccgtgaagcagctgaaagaggactacttcaagaaaatcgagtgcttcgactccgtggaaatctccggcgtggaagatagattcaacgcctccctgggcacataccacgatctgctgaaaattatcaaggacaaggacttcctggataacgaagagaacgaggacattctggaagatatcgtgctgaccctgacactgtttgaggaccgcgagatgatcgaggaaaggctgaaaacctacgctcacctgttcgacgacaaagtgatgaagcagctgaagagaaggcggtacaccggctggggcaggctgagcagaaagctgatcaacggcatcagagacaagcagagcggcaagacaatcctggatttcctgaagtccgacggcttcgccaaccggaacttcatgcagctgatccacgacgacagcctgacattcaaagaggacatccagaaagcccaggtgtccggccagggcgactctctgcacgagcatatcgctaacctggccggcagccccgctatcaagaagggcatcctgcagacagtgaaggtggtggacgagctcgtgaaagtgatgggcagacacaagcccgagaacatcgtgatcgagatggctagagagaaccagaccacccagaagggacagaagaactcccgcgagaggatgaagagaatcgaagagggcatcaaagagctgggcagccagatcctgaaagaacaccccgtggaaaacacccagctgcagaacgagaagctgtacctgtactacctgcagaatggccgggatatgtacgtggaccaggaactggacatcaacagactgtccgactacgatgtggaccatatcgtgcctcagagctttctgaaggacgactccatcgataacaaagtgctgactcggagcgacaagaacagaggcaagagcgacaacgtgccctccgaagaggtcgtgaagaagatgaagaactactggcgacagctgctgaacgccaagctgattacccagaggaagttcgataacctgaccaaggccgagagaggcggcctgagcgagctggataaggccggcttcatcaagaggcagctggtggaaaccagacagatcacaaagcacgtggcacagatcctggactcccggatgaacactaagtacgacgaaaacgataagctgatccgggaagtgaaagtgatcaccctgaagtccaagctggtgtccgatttccggaaggatttccagttttacaaagtgcgcgagatcaacaactaccaccacgcccacgacgcctacctgaacgccgtcgtgggaaccgccctgatcaaaaagtaccctaagctggaaagcgagttcgtgtacggcgactacaaggtgtacgacgtgcggaagatgatcgccaagagcgagcaggaaatcggcaaggctaccgccaagtacttcttctacagcaacatcatgaactttttcaagaccgaaatcaccctggccaacggcgagatcagaaagcgccctctgatcgagacaaacggcgaaaccggggagatcgtgtgggataagggcagagacttcgccacagtgcgaaaggtgctgagcatgccccaagtgaatatcgtgaaaaagaccgaggtgcagacaggcggcttcagcaaagagtctatcctgcccaagaggaacagcgacaagctgatcgccagaaagaaggactgggaccccaagaagtacggcggcttcgacagccctaccgtggcctactctgtgctggtggtggctaaggtggaaaagggcaagtccaagaaactgaagagtgtgaaagagctgctggggatcaccatcatggaaagaagcagctttgagaagaaccctatcgactttctggaagccaagggctacaaagaagtgaaaaaggacctgatcatcaagctgcctaagtactccctgttcgagctggaaaacggcagaaagagaatgctggcctctgccggcgaactgcagaagggaaacgagctggccctgcctagcaaatatgtgaacttcctgtacctggcctcccactatgagaagctgaagggcagccctgaggacaacgaacagaaacagctgtttgtggaacagcataagcactacctggacgagatcatcgagcagatcagcgagttctccaagagagtgatcctggccgacgccaatctggacaaggtgctgtctgcctacaacaagcacagggacaagcctatcagagagcaggccgagaatatcatccacctgttcaccctgacaaacctgggcgctcctgccgccttcaagtactttgacaccaccatcgaccggaagaggtacaccagcaccaaagaggtgctggacgccaccctgatccaccagagcatcaccggcctgtacgagacaagaatcgacctgtctcagctgggaggcgacaagagacctgccgccactaagaaggccggacaggccaaaaagaagaagggaagcggagccactaacttctccctgttgaaacaagcaggggatgtcgaagagaatcccgggccagtgagcaagggcgaggagctgttcaccggggtggtgcccatcctggtcgagctggacggcgacgtaaacggccacaagttcagcgtgtccggcgagggcgagggcgatgccacctacggcaagctgaccctgaagttcatctgcaccaccggcaagctgcccgtgccctggcccaccctcgtgaccaccctgacctacggcgtgcagtgcttcagccgctaccccgaccacatgaagcagcacgacttcttcaagtccgccatgcccgaaggctacgtccaggagcgcaccatcttcttcaaggacgacggcaactacaagacccgcgccgaggtgaagttcgagggcgacaccctggtgaaccgcatcgagctgaagggcatcgacttcaaggaggacggcaacatcctggggcacaagctggagtacaactacaacagccacaacgtctatatcatggccgacaagcagaagaacggcatcaaggtgaacttcaagatccgccacaacatcgaggacggcagcgtgcagctcgccgaccactaccagcagaacacccccatcggcgacggccccgtgctgctgcccgacaaccactacctgagcacccagtccgccctgagcaaagaccccaacgagaagcgcgatcacatggtcctgctggagttcgtgaccgccgccgggatcactctcggcatggacgagctgtacaagtaaacgcgtatgcatggccggccctgcaggaattcgatatcaagcttatcgataatcaacctctggattacaaaatttgtgaaagattgactggtattcttaactatgttgctccttttacgctatgtggatacgctgctttaatgcctttgtatcatgctattgcttcccgtatggctttcattttctcctccttgtataaatcctggttgctgtctctttatgaggagttgtggcccgttgtcaggcaacgtggcgtggtgtgcactgtgtttgctgacgcaacccccactggttggggcattgccaccacctgtcagctcctttccgggactttcgctttccccctccctattgccacggcggaactcatcgccgcctgccttgcccgctgctggacaggggctcggctgttgggcactgacaattccgtggtgttgtcggggaaatcatcgtcctttccttggctgctcgcctgtgttgccacctggattctgcgcgggacgtccttctgctacgtcccttcggccctcaatccagcggaccttccttcccgcggcctgctgccggctctgcggcctcttccgcgtcttcgccttcgccctcagacgagtcggatctccctttgggccgcctccccgcatcgcgacctcgacctcgactgtgccttctagttgccagccatctgttgtttgcccctcccccgtgccttccttgaccctggaaggtgccactcccactgtcctttcctaataaaatgaggaaattgcatcgcattgtctgagtaggtgtcattctattctggggggtggggtggggcaggacagcaagggggaggattgggaagacaatggcaggcatgctggggaactagtggtgccagggcgtgcccttgggctccccgggcgcggcggccatcgctcgagtaaaattggagggacaagacttcccacagattttcggttttgtcgggaagttttttaataggggcaaataaggaaaatgggaggataggtagtcatctggggttttatgcagcaaaactacaggttattattgcttgtgatccgc

SEQ ID NO: 15 - DNA, 8222 bp, Artificial Sequence
  Synthetic
  misc_feature (1)..(170): Mouse Rosa26 Upstream
  misc_feature (195)..(1913): CAGG Promoter
  misc_feature (1996)..(2029): LoxP
  misc_feature (2124)..(2133): Kozak
  misc_feature (2133)..(2198): 3xFLAG
  misc_feature (2199)..(6371): Cas9
  misc_feature (2208)..(2228): Monopartite NLS
  misc_feature (6324)..(6371): Bipartite NLS
  misc_feature (6372)..(6437): P2A
  misc_feature (6438)..(7151): eGFP
  misc_feature (7201)..(7797): WPRE
  misc_feature (7798)..(8013): bGH PolyA
  misc_feature (8073)..(8222): Mouse Rosa26 Downstream
ctgcagtggagtaggcggggagaaggccgcacccttctccggaggggggaggggagtgttgcaatacctttctgggagttctctgctgcctcctggcttctgaggaccgccctgggcctgggagaatcccttccccctcttccctcgtgatctgcaactccagtctttctccttaattaaggcctccaaggcctactagttattaatagtaatcaattacggggtcattagttcatagcccatatatggagttccgcgttacataacttacggtaaatggcccgcctggctgaccgcccaacgacccccgcccattgacgtcaataatgacgtatgttcccatagtaacgccaatagggactttccattgacgtcaatgggtggagtatttacggtaaactgcccacttggcagtacatcaagtgtatcatatgccaagtacgccccctattgacgtcaatgacggtaaatggcccgcctggcattatgcccagtacatgaccttatgggactttcctacttggcagtacatctacgtattagtcatcgctattaccatggtcgaggtgagccccacgttctgcttcactctccccatctcccccccctccccacccccaattttgtatttatttattttttaattattttgtgcagcgatgggggcggggggggggggggggcgcgcgccaggcggggcggggcggggcgaggggcggggcggggcgaggcggagaggtgcggcggcagccaatcagagcggcgcgctccgaaagtttccttttatggcgaggcggcggcggcggcggccctataaaaagcgaagcgcgcggcgggcggggagtcgctgcgacgctgccttcgccccgtgccccgctccgccgccgcctcgcgccgcccgccccggctctgactgaccgcgttactcccacaggtgagcgggcgggacggcccttctcctccgggctgtaattagcgcttggtttaatgacggcttgtttcttttctgtggctgcgtgaaagccttgaggggctccgggagggccctttgtgcggggggagcggctcggggggtgcgtgcgtgtgtgtgtgcgtggggagcgccgcgtgcggctccgcgctgcccggcggctgtgagcgctgcgggcgcggcgcggggctttgtgcgctccgcagtgtgcgcgaggggagcgcggccgggggcggtgccccgcggtgcggggggggctgcgaggggaacaaaggctgcgtgcggggtgtgtgcgtgggggggtgagcagggggtgtgggcgcgtcggtcgggctgcaaccccccctgcacccccctccccgagttgctgagcacggcccggcttcgggtgcggggctccgtacggggcgtggcgcggggctcgccgtgccgggcggggggtggcggcaggtgggggtgccgggcggggcggggccgcctcgggccggggagggctcgggggaggggcgcggcggcccccggagcgccggcggctgtcgaggcgcggcgagccgcagccattgccttttatggtaatcgtgcgagagggcgcagggacttcctttgtcccaaatctgtgcggagccgaaatctgggaggcgccgccgcaccccctctagcgggcgcggggcgaagcggtgcggcgccggcaggaaggaaatgggcggggagggccttcgtgcgtcgccgcgccgccgtccccttctccctctccagcctcggggctgtccgcggggggacggctgccttcgggggggacggggcagggcggggttcggcttctggcgtgtgaccggcggctctagagcctctgctaaccatgttcatgccttcttctttttcctacagctcctgggcaacgtgctggttattgtgctgtctcatcattttggcaaagaattcgctaggagaattgatttgataccgcgggccctaagtcgacatttaaatcatttaaatccactagtggatccggaacccttaatataacttcgtataatgtatgctatacgaagttattaggtccctcgacctgcagcccaagctagtgcccgggtaggtccctcgacctgcagcccaagctagatcgaattcggccggccttcgaacacgtgccaccatggactataaggaccacgacggagactacaaggatcatgatattgattacaaagacgatgacgataagatggacaagcccaagaaaaagcggaaagtgaagtacagcatcggcctggacatcggcaccaactctgtgggctgggccgtgatcaccgacgagtacaaggtgcccagcaagaaattcaaggtgctgggcaacaccgacaggcacagcatcaagaagaacctgatcggcgccctgctgttcgacagcggcgaaacagccgaggccaccagactgaagagaaccgccagaagaagatacaccaggcggaagaacaggatctgctatctgcaagagatcttcagcaacgagatggccaaggtggacgacagcttcttccacagactggaagagtccttcctggtggaagaggacaagaagcacgagagacaccccatcttcggcaacatcgtggacgaggtggcctaccacgagaagtaccccaccatctaccacctgagaaagaaactggtggacagcaccgacaaggccgacctgagactgatctacctggccctggcccacatgatcaagttcagaggccacttcctgatcgagggcgacctgaaccccgacaacagcgacgtggacaagctgttcatccagctggtgcagacctacaaccagctgttcgaggaaaaccccatcaacgccagcggcgtggacgccaaggctatcctgtctgccagactgagcaagagcagaaggctggaaaatctgatcgcccagctgcccggcgagaagaagaacggcctgttcggcaacctgattgccctgagcctgggcctgacccccaacttcaagagcaacttcgacctggccgaggatgccaaactgcagctgagcaaggacacctacgacgacgacctggacaacctgctggcccagatcggcgaccagtacgccgacctgttcctggccgccaagaacctgtctgacgccatcctgctgagcgacatcctgagagtgaacaccgagatcaccaaggcccccctgagcgcctctatgatcaagagatacgacgagcaccaccaggacctgaccctgctgaaagctctcgtgcggcagcagctgcctgagaagtacaaagaaatcttcttcgaccagagcaagaacggctacgccggctacatcgatggcggcgctagccaggaagagttctacaagttcatcaagcccatcctggaaaagatggacggcaccgaggaactgctcgtgaagctgaacagagaggacctgctgagaaagcagagaaccttcgacaacggcagcatcccccaccagatccacctgggagagctgcacgctatcctgagaaggcaggaagatttttacccattcctgaaggacaaccgggaaaagatcgagaagatcctgaccttcaggatcccctactacgtgggccccctggccagaggcaacagcagattcgcctggatgaccagaaagagcgaggaaaccatcaccccctggaacttcgaggaagtggtggacaagggcgccagcgcccagagcttcatcgagagaatgacaaacttcgataagaacctgcccaacgagaaggtgctgcccaagcacagcctgctgtacgagtacttcaccgtgtacaacgagctgaccaaagtgaaatacgtgaccgagggaatgagaaagcccgccttcctgagcggcgagcagaaaaaggccatcgtggacctgctgttcaagaccaacagaaaagtgaccgtgaagcagctgaaagaggactacttcaagaaaatcgagtgcttcgactccgtggaaatctccggcgtggaagatagattcaacgcctccctgggcacataccacgatctgctgaaaattatcaaggacaaggacttcctggataacgaagagaacgaggacattctggaagatatcgtgctgaccctgacactgtttgaggaccgcgagatgatcgaggaaaggctgaaaacctacgctcacctgttcgacgacaaagtgatgaagcagctgaagagaaggcggtacaccggctggggcaggctgagcagaaagctgatcaacggcatcagagacaagcagagcggcaagacaatcctggatttcctgaagtccgacggcttcgccaaccggaacttcatgcagctgatccacgacgacagcctgacattcaaagaggacatccagaaagcccaggtgtccggccagggcgactctctgcacgagcatatcgctaacctggccggcagccccgctatcaagaagggcatcctgcagacagtgaaggtggtggacgagctcgtgaaagtgatgggcagacacaagcccgagaacatcgtgatcgagatggctagagagaaccagaccacccagaagggacagaagaactcccgcgagaggatgaagagaatcgaagagggcatcaaagagctgggcagccagatcctgaaagaacaccccgtggaaaacacccagctgcagaacgagaagctgtacctgtactacctgcagaatggccgggatatgtacgtggaccaggaactggacatcaacagactgtccgactacgatgtggaccatatcgtgcctcagagctttctgaaggacgactccatcgataacaaagtgctgactcggagcgacaagaacagaggcaagagcgacaacgtgccctccgaagaggtcgtgaagaagatgaagaactactggcgacagctgctgaacgccaagctgattacccagaggaagttcgataacctgaccaaggccgagagaggcggcctgagcgagctggataaggccggcttcatcaagaggcagctggtggaaaccagacagatcacaaagcacgtggcacagatcctggactcccggatgaacactaagtacgacgaaaacgataagctgatccgggaagtgaaagtgatcaccctgaagtccaagctggtgtccgatttccggaaggatttccagttttacaaagtgcgcgagatcaacaactaccaccacgcccacgacgcctacctgaacgccgtcgtgggaaccgccctgatcaaaaagtaccctaagctggaaagcgagttcgtgtacggcgactacaaggtgtacgacgtgcggaagatgatcgccaagagcgagcaggaaatcggcaaggctaccgccaagtacttcttctacagcaacatcatgaactttttcaagaccgaaatcaccctggccaacggcgagatcagaaagcgccctctgatcgagacaaacggcgaaaccggggagatcgtgtgggataagggcagagacttcgccacagtgcgaaaggtgctgagcatgccccaagtgaatatcgtgaaaaagaccgaggtgcagacaggcggcttcagcaaagagtctatcctgcccaagaggaacagcgacaagctgatcgccagaaagaaggactgggaccccaagaagtacggcggcttcgacagccctaccgtggcctactctgtgctggtggtggctaaggtggaaaagggcaagtccaagaaactgaagagtgtgaaagagctgctggggatcaccatcatggaaagaagcagctttgagaagaaccctatcgactttctggaagccaagggctacaaagaagtgaaaaaggacctgatcatcaagctgcctaagtactccctgttcgagctggaaaacggcagaaagagaatgctggcctctgccggcgaactgcagaagggaaacgagctggccctgcctagcaaatatgtgaacttcctgtacctggcctcccactatgagaagctgaagggcagccctgaggacaacgaacagaaacagctgtttgtggaacagcataagcactacctggacgagatcatcgagcagatcagcgagttctccaagagagtgatcctggccgacgccaatctggacaaggtgctgtctgcctacaacaagcacagggacaagcctatcagagagcaggccgagaatatcatccacctgttcaccctgacaaacctgggcgctcctgccgccttcaagtactttgacaccaccatcgaccggaagaggtacaccagcaccaaagaggtgctggacgccaccctgatccaccagagcatcaccggcctgtacgagacaagaatcgacctgtctcagctgggaggcgacaagagacctgccgccactaagaaggccggacaggccaaaaagaagaagggaagcggagccactaacttctccctgttgaaacaagcaggggatgtcgaagagaatcccgggccagtgagcaagggcgaggagctgttcaccggggtggtgcccatcctggtcgagctggacggcgacgtaaacggccacaagttcagcgtgtccggcgagggcgagggcgatgccacctacggcaagctgaccctgaagttcatctgcaccaccggcaagctgcccgtgccctggcccaccctcgtgaccaccctgacctacggcgtgcagtgcttcagccgctaccccgaccacatgaagcagcacgacttcttcaagtccgccatgcccgaaggctacgtccaggagcgcaccatcttcttcaaggacgacggcaactacaagacccgcgccgaggtgaagttcgagggcgacaccctggtgaaccgcatcgagctgaagggcatcgacttcaaggaggacggcaacatcctggggcacaagctggagtacaactacaacagccacaacgtctatatcatggccgacaagcagaagaacggcatcaaggtgaacttcaagatccgccacaacatcgaggacggcagcgtgcagctcgccgaccactaccagcagaacacccccatcggcgacggccccgtgctgctgcccgacaaccactacctgagcacccagtccgccctgagcaaagaccccaacgagaagcgcgatcacatggtcctgctggagttcgtgaccgccgccgggatcactctcggcatggacgagctgtacaagtaaacgcgtatgcatggccggccctgcaggaattcgatatcaagcttatcgataatcaacctctggattacaaaatttgtgaaagattgactggtattcttaactatgttgctccttttacgctatgtggatacgctgctttaatgcctttgtatcatgctattgcttcccgtatggctttcattttctcctccttgtataaatcctggttgctgtctctttatgaggagttgtggcccgttgtcaggcaacgtggcgtggtgtgcactgtgtttgctgacgcaacccccactggttggggcattgccaccacctgtcagctcctttccgggactttcgctttccccctccctattgccacggcggaactcatcgccgcctgccttgcccgctgctggacaggggctcggctgttgggcactgacaattccgtggtgttgtcggggaaatcatcgtcctttccttggctgctcgcctgtgttgccacctggattctgcgcgggacgtccttctgctacgtcccttcggccctcaatccagcggaccttccttcccgcggcctgctgccggctctgcggcctcttccgcgtcttcgccttcgccctcagacgagtcggatctccctttgggccgcctccccgcatcgcgacctcgacctcgactgtgccttctagttgccagccatctgttgtttgcccctcccccgtgccttccttgaccctggaaggtgccactcccactgtcctttcctaataaaatgaggaaattgcatcgcattgtctgagtaggtgtcattctattctggggggtggggtggggcaggacagcaagggggaggattgggaagacaatggcaggcatgctggggaactagtggtgccagggcgtgcccttgggctccccgggcgcggcggccatcgctcgagtaaaattggagggacaagacttcccacagattttcggttttgtcgggaagttttttaataggggcaaataaggaaaatgggaggataggtagtcatctggggttttatgcagcaaaactacaggttattattgcttgtgatccgc

SEQ ID NO: 16 - protein, 1673 aa, Artificial Sequence
  Synthetic
  MISC_FEATURE (1)..(22): 3xFLAG
  MISC_FEATURE (23)..(1413): Cas9
  MISC_FEATURE (1414)..(1435): P2A
  MISC_FEATURE (1436)..(1673): eGFP
DYKDHDGDYKDHDIDYKDDDDKMDKPKKKRKVKYSIGLDIGTNSVGWAVITDEYKVPSKKFKVLGNTDRHSIKKNLIGALLFDSGETAEATRLKRTARRRYTRRKNRICYLQEIFSNEMAKVDDSFFHRLEESFLVEEDKKHERHPIFGNIVDEVAYHEKYPTIYHLRKKLVDSTDKADLRLIYLALAHMIKFRGHFLIEGDLNPDNSDVDKLFIQLVQTYNQLFEENPINASGVDAKAILSARLSKSRRLENLIAQLPGEKKNGLFGNLIALSLGLTPNFKSNFDLAEDAKLQLSKDTYDDDLDNLLAQIGDQYADLFLAAKNLSDAILLSDILRVNTEITKAPLSASMIKRYDEHHQDLTLLKALVRQQLPEKYKEIFFDQSKNGYAGYIDGGASQEEFYKFIKPILEKMDGTEELLVKLNREDLLRKQRTFDNGSIPHQIHLGELHAILRRQEDFYPFLKDNREKIEKILTFRIPYYVGPLARGNSRFAWMTRKSEETITPWNFEEVVDKGASAQSFIERMTNFDKNLPNEKVLPKHSLLYEYFTVYNELTKVKYVTEGMRKPAFLSGEQKKAIVDLLFKTNRKVTVKQLKEDYFKKIECFDSVEISGVEDRFNASLGTYHDLLKIIKDKDFLDNEENEDILEDIVLTLTLFEDREMIEERLKTYAHLFDDKVMKQLKRRRYTGWGRLSRKLINGIRDKQSGKTILDFLKSDGFANRNFMQLIHDDSLTFKEDIQKAQVSGQGDSLHEHIANLAGSPAIKKGILQTVKVVDELVKVMGRHKPENIVIEMARENQTTQKGQKNSRERMKRIEEGIKELGSQILKEHPVENTQLQNEKLYLYYLQNGRDMYVDQELDINRLSDYDVDHIVPQSFLKDDSIDNKVLTRSDKNRGKSDNVPSEEVVKKMKNYWRQLLNAKLITQRKFDNLTKAERGGLSELDKAGFIKRQLVETRQITKHVAQILDSRMNTKYDENDKLIREVKVITLKSKLVSDFRKDFQFYKVREINNYHHAHDAYLNAVVGTALIKKYPKLESEFVYGDYKVYDVRKMIAKSEQEIGKATAKYFFYSNIMNFFKTEITLANGEIRKRPLIETNGETGEIVWDKGRDFATVRKVLSMPQVNIVKKTEVQTGGFSKESILPKRNSDKLIARKKDWDPKKYGGFDSPTVAYSVLVVAKVEKGKSKKLKSVKELLGITIMERSSFEKNPIDFLEAKGYKEVKKDLIIKLPKYSLFELENGRKRMLASAGELQKGNELALPSKYVNFLYLASHYEKLKGSPEDNEQKQLFVEQHKHYLDEIIEQISEFSKRVILADANLDKVLSAYNKHRDKPIREQAENIIHLFTLTNLGAPAAFKYFDTTIDRKRYTSTKEVLDATLIHQSITGLYETRIDLSQLGGDKRPAATKKAGQAKKKKGSGATNFSLLKQAGDVEENPGPVSKGEELFTGVVPILVELDGDVNGHKFSVSGEGEGDATYGKLTLKFICTTGKLPVPWPTLVTTLTYGVQCFSRYPDHMKQHDFFKSAMPEGYVQERTIFFKDDGNYKTRAEVKFEGDTLVNRIELKGIDFKEDGNILGHKLEYNYNSHNVYIMADKQKNGIKVNFKIRHNIEDGSVQLADHYQQNTPIGDGPVLLPDNHYLSTQSALSKDPNEKRDHMVLLEFVTAAGITLGMDELYK

SEQ ID NO: 17 - DNA, 7207 bp, Artificial Sequence
  Synthetic
  misc_feature (1)..(170): Mouse Rosa26 Upstream
  misc_feature (300)..(333): LoxP
  misc_feature (424)..(2489): Neo-PolyA
  misc_feature (2517)..(2550): LoxP
  misc_feature (2599)..(2608): Kozak
  misc_feature (2605)..(6777): Cas9
  misc_feature (2614)..(2634): Monopartite NLS
  misc_feature (6730)..(6777): Bipartite NLS
  misc_feature (6783)..(6998): bGH PolyA
  misc_feature (7058)..(7207): Mouse Rosa26 Downstream
ctgcagtggagtaggcggggagaaggccgcacccttctccggaggggggaggggagtgttgcaatacctttctgggagttctctgctgcctcctggcttctgaggaccgccctgggcctgggagaatcccttccccctcttccctcgtgatctgcaactccagtctttctagttgaccagctcggcggtgacctgcacgtctagggcgcagtagtccagggtttccttgatgatgtcatacttatcctgtcccttttttttccacagggcgcgccactagtggatccggaacccttaatataacttcgtataatgtatgctatacgaagttattaggtccctcgacctgcaggaattgttgacaattaatcatcggcatagtatatcggcatagtataatacgacaaggtgaggaactaaaccatgggatcggccattgaacaagatggattgcacgcaggttctccggccgcttgggtggagaggctattcggctatgactgggcacaacagacaatcggctgctctgatgccgccgtgttccggctgtcagcgcaggggcgcccggttctttttgtcaagaccgacctgtccggtgccctgaatgaactgcaggacgaggcagcgcggctatcgtggctggccacgacgggcgttccttgcgcagctgtgctcgacgttgtcactgaagcgggaagggactggctgctattgggcgaagtgccggggcaggatctcctgtcatctcaccttgctcctgccgagaaagtatccatcatggctgatgcaatgcggcggctgcatacgcttgatccggctacctgcccattcgaccaccaagcgaaacatcgcatcgagcgagcacgtactcggatggaagccggtcttgtcgatcaggatgatctggacgaagagcatcaggggctcgcgccagccgaactgttcgccaggctcaaggcgcgcatgcccgacggcgatgatctcgtcgtgacccatggcgatgcctgcttgccgaatatcatggtggaaaatggccgcttttctggattcatcgactgtggccggctgggtgtggcggaccgctatcaggacatagcgttggctacccgtgatattgctgaagagcttggcggcgaatgggctgaccgcttcctcgtgctttacggtatcgccgctcccgattcgcagcgcatcgccttctatcgccttcttgacgagttcttctgaggggatccgctgtaagtctgcagaaattgatgatctattaaacaataaagatgtccactaaaatggaagtttttcctgtcatactttgttaagaagggtgagaacagagtacctacattttgaatggaaggattggagctacgggggtgggggtggggtgggattagataaatgcctgctctttactgaaggctctttactattgctttatgataatgtttcatagttggatatcataatttaaacaagcaaaaccaaattaagggccagctcattcctcccactcatgatctatagatctatagatctctcgtgggatcattgtttttctcttgattcccactttgtggttctaagtactgtggtttccaaatgtgtcagtttcatagcctgaagaacgagatcagcagcctctgttccacatacacttcattctcagtattgttttgccaagttctaattccatcagaagcttgcagatctgcgactctagaggatctgcgactctagaggatcataatcagccataccacatttgtagaggttttacttgctttaaaaaacctcccacacctccccctgaacctgaaacataaaatgaatgcaattgttgttgttaacttgtttattgcagcttataatggttacaaataaagcaatagcatcacaaatttcacaaataaagcatttttttcactgcattctagttgtggtttgtccaaactcatcaatgtatcttatcatgtctggatctgcgactctagaggatcataatcagccataccacatttgtagaggttttacttgctttaaaaaacctcccacacctccccctgaacctgaaacataaaatgaatgcaattgttgttgttaacttgtttattgcagcttataatggttacaaataaagcaatagcatcacaaatttcacaaataaagcatttttttcactgcattctagttgtggtttgtccaaactcatcaatgtatcttatcatgtctggatctgcgactctagaggatcataatcagccataccacatttgtagaggttttacttgctttaaaaaacctcccacacctccccctgaacctgaaacataaaatgaatgcaattgttgttgttaacttgtttattgcagcttataatggttacaaataaagcaatagcatcacaaatttcacaaataaagcatttttttcactgcattctagttgtggtttgtccaaactcatcaatgtatcttatcatgtctggatccccatcaagctgatccggaacccttaatataacttcgtataatgtatgctatacgaagttattaggtccctcgacctgcagcccaagctagtgcccgggaattcgctagggccaccatggacaagcccaagaaaaagcggaaagtgaagtacagcatcggcctggacatcggcaccaactctgtgggctgggccgtgatcaccgacgagtacaaggtgcccagcaagaaattcaaggtgctgggcaacaccgacaggcacagcatcaagaagaacctgatcggcgccctgctgttcgacagcggcgaaacagccgaggccaccagactgaagagaaccgccagaagaagatacaccaggcggaagaacaggatctgctatctgcaagagatcttcagcaacgagatggccaaggtggacgacagcttcttccacagactggaagagtccttcctggtggaagaggacaagaagcacgagagacaccccatcttcggcaacatcgtggacgaggtggcctaccacgagaagtaccccaccatctaccacctgagaaagaaactggtggacagcaccgacaaggccgacctgagactgatctacctggccctggcccacatgatcaagttcagaggccacttcctgatcgagggcgacctgaaccccgacaacagcgacgtggacaagctgttcatccagctggtgcagacctacaaccagctgttcgaggaaaaccccatcaacgccagcggcgtggacgccaaggctatcctgtctgccagactgagcaagagcagaaggctggaaaatctgatcgcccagctgcccggcgagaagaagaacggcctgttcggcaacctgattgccctgagcctgggcctgacccccaacttcaagagcaacttcgacctggccgaggatgccaaactgcagctgagcaaggacacctacgacgacgacctggacaacctgctggcccagatcggcgaccagtacgccgacctgttcctggccgccaagaacctgtctgacgccatcctgctgagcgacatcctgagagtgaacaccgagatcaccaaggcccccctgagcgcctctatgatcaagagatacgacgagcaccaccaggacctgaccctgctgaaagctctcgtgcggcagcagctgcctgagaagtacaaagaaatcttcttcgaccagagcaagaacggctacgccggctacatcgatggcggcgctagccaggaagagttctacaagttcatcaagcccatcctggaaaagatggacggcaccgaggaactgctcgtgaagctgaacagagaggacctgctgagaaagcagagaaccttcgacaacggcagcatcccccaccagatccacctgggagagctgcacgctatcctgagaaggcaggaagatttttacccattcctgaaggacaaccgggaaaagatcgagaagatcctgaccttcaggatcccctactacgtgggccccctggccagaggcaacagcagattcgcctggatgaccagaaagagcgaggaaaccatcaccccctggaacttcgaggaagtggtggacaagggcgccagcgcccagagcttcatcgagagaatgacaaacttcgataagaacctgcccaacgagaaggtgctgcccaagcacagcctgctgtacgagtacttcaccgtgtacaacgagctgaccaaagtgaaatacgtgaccgagggaatgagaaagcccgccttcctgagcggcgagcagaaaaaggccatcgtggacctgctgttcaagaccaacagaaaagtgaccgtgaagcagctgaaagaggactacttcaagaaaatcgagtgcttcgactccgtggaaatctccggcgtggaagatagattcaacgcctccctgggcacataccacgatctgctgaaaattatcaaggacaaggacttcctggataacgaagagaacgaggacattctggaagatatcgtgctgaccctgacactgtttgaggaccgcgagatgatcgaggaaaggctgaaaacctacgctcacctgttcgacgacaaagtgatgaagcagctgaagagaaggcggtacaccggctggggcaggctgagcagaaagctgatcaacggcatcagagacaagcagagcggcaagacaatcctggatttcctgaagtccgacggcttcgccaaccggaacttcatgcagctgatccacgacgacagcctgacattcaaagaggacatccagaaagcccaggtgtccggccagggcgactctctgcacgagcatatcgctaacctggccggcagccccgctatcaagaagggcatcctgcagacagtgaaggtggtggacgagctcgtgaaagtgatgggcagacacaagcccgagaacatcgtgatcgagatggctagagagaaccagaccacccagaagggacagaagaactcccgcgagaggatgaagagaatcgaagagggcatcaaagagctgggcagccagatcctgaaagaacaccccgtggaaaacacccagctgcagaacgagaagctgtacctgtactacctgcagaatggccgggatatgtacgtggaccaggaactggacatcaacagactgtccgactacgatgtggaccatatcgtgcctcagagctttctgaaggacgactccatcgataacaaagtgctgactcggagcgacaagaacagaggcaagagcgacaacgtgccctccgaagaggtcgtgaagaagatgaagaactactggcgacagctgctgaacgccaagctgattacccagaggaagttcgataacctgaccaaggccgagagaggcggcctgagcgagctggataaggccggcttcatcaagaggcagctggtggaaaccagacagatcacaaagcacgtggcacagatcctggactcccggatgaacactaagtacgacgaaaacgataagctgatccgggaagtgaaagtgatcaccctgaagtccaagctggtgtccgatttccggaaggatttccagttttacaaagtgcgcgagatcaacaactaccaccacgcccacgacgcctacctgaacgccgtcgtgggaaccgccctgatcaaaaagtaccctaagctggaaagcgagttcgtgtacggcgactacaaggtgtacgacgtgcggaagatgatcgccaagagcgagcaggaaatcggcaaggctaccgccaagtacttcttctacagcaacatcatgaactttttcaagaccgaaatcaccctggccaacggcgagatcagaaagcgccctctgatcgagacaaacggcgaaaccggggagatcgtgtgggataagggcagagacttcgccacagtgcgaaaggtgctgagcatgccccaagtgaatatcgtgaaaaagaccgaggtgcagacaggcggcttcagcaaagagtctatcctgcccaagaggaacagcgacaagctgatcgccagaaagaaggactgggaccccaagaagtacggcggcttcgacagccctaccgtggcctactctgtgctggtggtggctaaggtggaaaagggcaagtccaagaaactgaagagtgtgaaagagctgctggggatcaccatcatggaaagaagcagctttgagaagaaccctatcgactttctggaagccaagggctacaaagaagtgaaaaaggacctgatcatcaagctgcctaagtactccctgttcgagctggaaaacggcagaaagagaatgctggcctctgccggcgaactgcagaagggaaacgagctggccctgcctagcaaatatgtgaacttcctgtacctggcctcccactatgagaagctgaagggcagccctgaggacaacgaacagaaacagctgtttgtggaacagcataagcactacctggacgagatcatcgagcagatcagcgagttctccaagagagtgatcctggccgacgccaatctggacaaggtgctgtctgcctacaacaagcacagggacaagcctatcagagagcaggccgagaatatcatccacctgttcaccctgacaaacctgggcgctcctgccgccttcaagtactttgacaccaccatcgaccggaagaggtacaccagcaccaaagaggtgctggacgccaccctgatccaccagagcatcaccggcctgtacgagacaagaatcgacctgtctcagctgggaggcgacaagagacctgccgccactaagaaggccggacaggccaaaaagaagaagtgagtcgacctcgacctcgactgtgccttctagttgccagccatctgttgtttgcccctcccccgtgccttccttgaccctggaaggtgccactcccactgtcctttcctaataaaatgaggaaattgcatcgcattgtctgagtaggtgtcattctattctggggggtggggtggggcaggacagcaagggggaggattgggaagacaatggcaggcatgctggggaactagtggtgccagggcgtgcccttgggctccccgggcgcggcggccatcgctcgagtaaaattggagggacaagacttcccacagattttcggttttgtcgggaagttttttaataggggcaaataaggaaaatgggaggataggtagtcatctggggttttatgcagcaaaactacaggttattattgcttgtgatccgc

SEQ ID NO: 18 - DNA, 4990 bp, Artificial Sequence
  Synthetic
  misc_feature (1)..(170): Mouse Rosa26 Upstream
  misc_feature (300)..(333): LoxP
  misc_feature (382)..(391): Kozak
  misc_feature (388)..(4560): Cas9
  misc_feature (397)..(417): Monopartite NLS
  misc_feature (4513)..(4560): Bipartite NLS
  misc_feature (4566)..(4781): bGH PolyA
  misc_feature (4841)..(4990): Mouse Rosa26 Downstream
ctgcagtggagtaggcggggagaaggccgcacccttctccggaggggggaggggagtgttgcaatacctttctgggagttctctgctgcctcctggcttctgaggaccgccctgggcctgggagaatcccttccccctcttccctcgtgatctgcaactccagtctttctagttgaccagctcggcggtgacctgcacgtctagggcgcagtagtccagggtttccttgatgatgtcatacttatcctgtcccttttttttccacagggcgcgccactagtggatccggaacccttaatataacttcgtataatgtatgctatacgaagttattaggtccctcgacctgcagcccaagctagtgcccgggaattcgctagggccaccatggacaagcccaagaaaaagcggaaagtgaagtacagcatcggcctggacatcggcaccaactctgtgggctgggccgtgatcaccgacgagtacaaggtgcccagcaagaaattcaaggtgctgggcaacaccgacaggcacagcatcaagaagaacctgatcggcgccctgctgttcgacagcggcgaaacagccgaggccaccagactgaagagaaccgccagaagaagatacaccaggcggaagaacaggatctgctatctgcaagagatcttcagcaacgagatggccaaggtggacgacagcttcttccacagactggaagagtccttcctggtggaagaggacaagaagcacgagagacaccccatcttcggcaacatcgtggacgaggtggcctaccacgagaagtaccccaccatctaccacctgagaaagaaactggtggacagcaccgacaaggccgacctgagactgatctacctggccctggcccacatgatcaagttcagaggccacttcctgatcgagggcgacctgaaccccgacaacagcgacgtggacaagctgttcatccagctggtgcagacctacaaccagctgttcgaggaaaaccccatcaacgccagcggcgtggacgccaaggctatcctgtctgccagactgagcaagagcagaaggctggaaaatctgatcgcccagctgcccggcgagaagaagaacggcctgttcggcaacctgattgccctgagcctgggcctgacccccaacttcaagagcaacttcgacctggccgaggatgccaaactgcagctgagcaaggacacctacgacgacgacctggacaacctgctggcccagatcggcgaccagtacgccgacctgttcctggccgccaagaacctgtctgacgccatcctgctgagcgacatcctgagagtgaacaccgagatcaccaaggcccccctgagcgcctctatgatcaagagatacgacgagcaccaccaggacctgaccctgctgaaagctctcgtgcggcagcagctgcctgagaagtacaaagaaatcttcttcgaccagagcaagaacggctacgccggctacatcgatggcggcgctagccaggaagagttctacaagttcatcaagcccatcctggaaaagatggacggcaccgaggaactgctcgtgaagctgaacagagaggacctgctgagaaagcagagaaccttcgacaacggcagcatcccccaccagatccacctgggagagctgcacgctatcctgagaaggcaggaagatttttacccattcctgaaggacaaccgggaaaagatcgagaagatcctgaccttcaggatcccctactacgtgggccccctggccagaggcaacagcagattcgcctggatgaccagaaagagcgaggaaaccatcaccccctggaacttcgaggaagtggtggacaagggcgccagcgcccagagcttcatcgagagaatgacaaacttcgataagaacctgcccaacgagaaggtgctgcccaagcacagcctgctgtacgagtacttcaccgtgtacaacgagctgaccaaagtgaaatacgtgaccgagggaatgagaaagcccgccttcctgagcggcgagcagaaaaaggccatcgtggacctgctgttcaagaccaacagaaaagtgaccgtgaagcagctgaaagaggactacttcaagaaaatcgagtgcttcgactccgtggaaatctccggcgtggaagatagattcaacgcctccctgggcacataccacgatctgctgaaaattatcaaggacaaggacttcctggataacgaagagaacgaggacattctggaagatatcgtgctgaccctgacactgtttgaggaccgcgagatgatcgaggaaaggctgaaaacctacgctcacctgttcgacgacaaagtgatgaagcagctgaagagaaggcggtacaccggctggggcaggctgagcagaaagctgatcaacggcatcagagacaagcagagcggcaagacaatcctggatttcctgaagtccgacggcttcgccaaccggaacttcatgcagctgatccacgacgacagcctgacattcaaagaggacatccagaaagcccaggtgtccggccagggcgactctctgcacgagcatatcgctaacctggccggcagccccgctatcaagaagggcatcctgcagacagtgaaggtggtggacgagctcgtgaaagtgatgggcagacacaagcccgagaacatcgtgatcgagatggctagagagaaccagaccacccagaagggacagaagaactcccgcgagaggatgaagagaatcgaagagggcatcaaagagctgggcagccagatcctgaaagaacaccccgtggaaaacacccagctgcagaacgagaagctgtacctgtactacctgcagaatggccgggatatgtacgtggaccaggaactggacatcaacagactgtccgactacgatgtggaccatatcgtgcctcagagctttctgaaggacgactccatcgataacaaagtgctgactcggagcgacaagaacagaggcaagagcgacaacgtgccctccgaagaggtcgtgaagaagatgaagaactactggcgacagctgctgaacgccaagctgattacccagaggaagttcgataacctgaccaaggccgagagaggcggcctgagcgagctggataaggccggcttcatcaagaggcagctggtggaaaccagacagatcacaaagcacgtggcacagatcctggactcccggatgaacactaagtacgacgaaaacgataagctgatccgggaagtgaaagtgatcaccctgaagtccaagctggtgtccgatttccggaaggatttccagttttacaaagtgcgcgagatcaacaactaccaccacgcccacgacgcctacctgaacgccgtcgtgggaaccgccctgatcaaaaagtaccctaagctggaaagcgagttcgtgtacggcgactacaaggtgtacgacgtgcggaagatgatcgccaagagcgagcaggaaatcggcaaggctaccgccaagtacttcttctacagcaacatcatgaactttttcaagaccgaaatcaccctggccaacggcgagatcagaaagcgccctctgatcgagacaaacggcgaaaccggggagatcgtgtgggataagggcagagacttcgccacagtgcgaaaggtgctgagcatgccccaagtgaatatcgtgaaaaagaccgaggtgcagacaggcggcttcagcaaagagtctatcctgcccaagaggaacagcgacaagctgatcgccagaaagaaggactgggaccccaagaagtacggcggcttcgacagccctaccgtggcctactctgtgctggtggtggctaaggtggaaaagggcaagtccaagaaactgaagagtgtgaaagagctgctggggatcaccatcatggaaagaagcagctttgagaagaaccctatcgactttctggaagccaagggctacaaagaagtgaaaaaggacctgatcatcaagctgcctaagtactccctgttcgagctggaaaacggcagaaagagaatgctggcctctgccggcgaactgcagaagggaaacgagctggccctgcctagcaaatatgtgaacttcctgtacctggcctcccactatgagaagctgaagggcagccctgaggacaacgaacagaaacagctgtttgtggaacagcataagcactacctggacgagatcatcgagcagatcagcgagttctccaagagagtgatcctggccgacgccaatctggacaaggtgctgtctgcctacaacaagcacagggacaagcctatcagagagcaggccgagaatatcatccacctgttcaccctgacaaacctgggcgctcctgccgccttcaagtactttgacaccaccatcgaccggaagaggtacaccagcaccaaagaggtgctggacgccaccctgatccaccagagcatcaccggcctgtacgagacaagaatcgacctgtctcagctgggaggcgacaagagacctgccgccactaagaaggccggacaggccaaaaagaagaagtgagtcgacctcgacctcgactgtgccttctagttgccagccatctgttgtttgcccctcccccgtgccttccttgaccctggaaggtgccactcccactgtcctttcctaataaaatgaggaaattgcatcgcattgtctgagtaggtgtcattctattctggggggtggggtggggcaggacagcaagggggaggattgggaagacaatggcaggcatgctggggaactagtggtgccagggcgtgcccttgggctccccgggcgcggcggccatcgctcgagtaaaattggagggacaagacttcccacagattttcggttttgtcgggaagttttttaataggggcaaataaggaaaatgggaggataggtagtcatctggggttttatgcagcaaaactacaggttattattgcttgtgatccgc

SEQ ID NO: 19 - protein, 1391 aa, Artificial Sequence
  Synthetic
MDKPKKKRKVKYSIGLDIGTNSVGWAVITDEYKVPSKKFKVLGNTDRHSIKKNLIGALLFDSGETAEATRLKRTARRRYTRRKNRICYLQEIFSNEMAKVDDSFFHRLEESFLVEEDKKHERHPIFGNIVDEVAYHEKYPTIYHLRKKLVDSTDKADLRLIYLALAHMIKFRGHFLIEGDLNPDNSDVDKLFIQLVQTYNQLFEENPINASGVDAKAILSARLSKSRRLENLIAQLPGEKKNGLFGNLIALSLGLTPNFKSNFDLAEDAKLQLSKDTYDDDLDNLLAQIGDQYADLFLAAKNLSDAILLSDILRVNTEITKAPLSASMIKRYDEHHQDLTLLKALVRQQLPEKYKEIFFDQSKNGYAGYIDGGASQEEFYKFIKPILEKMDGTEELLVKLNREDLLRKQRTFDNGSIPHQIHLGELHAILRRQEDFYPFLKDNREKIEKILTFRIPYYVGPLARGNSRFAWMTRKSEETITPWNFEEVVDKGASAQSFIERMTNFDKNLPNEKVLPKHSLLYEYFTVYNELTKVKYVTEGMRKPAFLSGEQKKAIVDLLFKTNRKVTVKQLKEDYFKKIECFDSVEISGVEDRFNASLGTYHDLLKIIKDKDFLDNEENEDILEDIVLTLTLFEDREMIEERLKTYAHLFDDKVMKQLKRRRYTGWGRLSRKLINGIRDKQSGKTILDFLKSDGFANRNFMQLIHDDSLTFKEDIQKAQVSGQGDSLHEHIANLAGSPAIKKGILQTVKVVDELVKVMGRHKPENIVIEMARENQTTQKGQKNSRERMKRIEEGIKELGSQILKEHPVENTQLQNEKLYLYYLQNGRDMYVDQELDINRLSDYDVDHIVPQSFLKDDSIDNKVLTRSDKNRGKSDNVPSEEVVKKMKNYWRQLLNAKLITQRKFDNLTKAERGGLSELDKAGFIKRQLVETRQITKHVAQILDSRMNTKYDENDKLIREVKVITLKSKLVSDFRKDFQFYKVREINNYHHAHDAYLNAVVGTALIKKYPKLESEFVYGDYKVYDVRKMIAKSEQEIGKATAKYFFYSNIMNFFKTEITLANGEIRKRPLIETNGETGEIVWDKGRDFATVRKVLSMPQVNIVKKTEVQTGGFSKESILPKRNSDKLIARKKDWDPKKYGGFDSPTVAYSVLVVAKVEKGKSKKLKSVKELLGITIMERSSFEKNPIDFLEAKGYKEVKKDLIIKLPKYSLFELENGRKRMLASAGELQKGNELALPSKYVNFLYLASHYEKLKGSPEDNEQKQLFVEQHKHYLDEIIEQISEFSKRVILADANLDKVLSAYNKHRDKPIREQAENIIHLFTLTNLGAPAAFKYFDTTIDRKRYTSTKEVLDATLIHQSITGLYETRIDLSQLGGDKRPAATKKAGQAKKKK

SEQ ID NO: 20 - DNA, 9673 bp, Artificial Sequence
  Synthetic
  misc_feature (1)..(170): Mouse Rosa26 Upstream
  misc_feature (205)..(1923): CAGG Promoter
  misc_feature (2006)..(2039): LoxP
  misc_feature (2130)..(4195): Neo-PolyA
  misc_feature (4223)..(4256): LoxP
  misc_feature (4351)..(4360): Kozak
  misc_feature (4360)..(4425): 3xFLAG
  misc_feature (4426)..(8598): Cas9
  misc_feature (4435)..(4455): Monopartite NLS
  misc_feature (8551)..(8598): Bipartite NLS
  misc_feature (8645)..(9241): WPRE
  misc_feature (9249)..(9464): bGH PolyA
  misc_feature (9524)..(9673): Mouse Rosa26 Downstream
ctgcagtggagtaggcggggagaaggccgcacccttctccggaggggggaggggagtgttgcaatacctttctgggagttctctgctgcctcctggcttctgaggaccgccctgggcctgggagaatcccttccccctcttccctcgtgatctgcaactccagtctttctccttaattaaacgcgtctggcctcgcgagtgtgtactagttattaatagtaatcaattacggggtcattagttcatagcccatatatggagttccgcgttacataacttacggtaaatggcccgcctggctgaccgcccaacgacccccgcccattgacgtcaataatgacgtatgttcccatagtaacgccaatagggactttccattgacgtcaatgggtggagtatttacggtaaactgcccacttggcagtacatcaagtgtatcatatgccaagtacgccccctattgacgtcaatgacggtaaatggcccgcctggcattatgcccagtacatgaccttatgggactttcctacttggcagtacatctacgtattagtcatcgctattaccatggtcgaggtgagccccacgttctgcttcactctccccatctcccccccctccccacccccaattttgtatttatttattttttaattattttgtgcagcgatgggggcggggggggggggggggcgcgcgccaggcggggcggggcggggcgaggggcggggcggggcgaggcggagaggtgcggcggcagccaatcagagcggcgcgctccgaaagtttccttttatggcgaggcggcggcggcggcggccctataaaaagcgaagcgcgcggcgggcggggagtcgctgcgacgctgccttcgccccgtgccccgctccgccgccgcctcgcgccgcccgccccggctctgactgaccgcgttactcccacaggtgagcgggcgggacggcccttctcctccgggctgtaattagcgcttggtttaatgacggcttgtttcttttctgtggctgcgtgaaagccttgaggggctccgggagggccctttgtgcggggggagcggctcggggggtgcgtgcgtgtgtgtgtgcgtggggagcgccgcgtgcggctccgcgctgcccggcggctgtgagcgctgcgggcgcggcgcggggctttgtgcgctccgcagtgtgcgcgaggggagcgcggccgggggcggtgccccgcggtgcggggggggctgcgaggggaacaaaggctgcgtgcggggtgtgtgcgtgggggggtgagcagggggtgtgggcgcgtcggtcgggctgcaaccccccctgcacccccctccccgagttgctgagcacggcccggcttcgggtgcggggctccgtacggggcgtggcgcggggctcgccgtgccgggcggggggtggcggcaggtgggggtgccgggcggggcggggccgcctcgggccggggagggctcgggggaggggcgcggcggcccccggagcgccggcggctgtcgaggcgcggcgagccgcagccattgccttttatggtaatcgtgcgagagggcgcagggacttcctttgtcccaaatctgtgcggagccgaaatctgggaggcgccgccgcaccccctctagcgggcgcggggcgaagcggtgcggcgccggcaggaaggaaatgggcggggagggccttcgtgcgtcgccgcgccgccgtccccttctccctctccagcctcggggctgtccgcggggggacggctgccttcgggggggacggggcagggcggggttcggcttctggcgtgtgaccggcggctctagagcctctgctaaccatgttcatgccttcttctttttcctacagctcctgggcaacgtgctggttattgtgctgtctcatcattttggcaaagaattcgctaggagaattgatttgataccgcgggccctaagtcgacatttaaatcatttaaatccactagtggatccggaacccttaatataacttcgtataatgtatgctatacgaagttattaggtccctcgacctgcaggaattgttgacaattaatcatcggcatagtatatcggcatagtataatacgacaaggtgaggaactaaaccatgggatcggccattgaacaagatggattgcacgcaggttctccggccgcttgggtggagaggctattcggctatgactgggcacaacagacaatcggctgctctgatgccgccgtgttccggctgtcagcgcaggggcgcccggttctttttgtcaagaccgacctgtccggtgccctgaatgaactgcaggacgaggcagcgcggctatcgtggctggccacgacgggcgttccttgcgcagctgtgctcgacgttgtcactgaagcgggaagggactggctgctattgggcgaagtgccggggcaggatctcctgtcatctcaccttgctcctgccgagaaagtatccatcatggctgatgcaatgcggcggctgcatacgcttgatccggctacctgcccattcgaccaccaagcgaaacatcgcatcgagcgagcacgtactcggatggaagccggtcttgtcgatcaggatgatctggacgaagagcatcaggggctcgcgccagccgaactgttcgccaggctcaaggcgcgcatgcccgacggcgatgatctcgtcgtgacccatggcgatgcctgcttgccgaatatcatggtggaaaatggccgcttttctggattcatcgactgtggccggctgggtgtggcggaccgctatcaggacatagcgttggctacccgtgatattgctgaagagcttggcggcgaatgggctgaccgcttcctcgtgctttacggtatcgccgctcccgattcgcagcgcatcgccttctatcgccttcttgacgagttcttctgaggggatccgctgtaagtctgcagaaattgatgatctattaaacaataaagatgtccactaaaatggaagtttttcctgtcatactttgttaagaagggtgagaacagagtacctacattttgaatggaaggattggagctacgggggtgggggtggggtgggattagataaatgcctgctctttactgaaggctctttactattgctttatgataatgtttcatagttggatatcataatttaaacaagcaaaaccaaattaagggccagctcattcctcccactcatgatctatagatctatagatctctcgtgggatcattgtttttctcttgattcccactttgtggttctaagtactgtggtttccaaatgtgtcagtttcatagcctgaagaacgagatcagcagcctctgttccacatacacttcattctcagtattgttttgccaagttctaattccatcagaagcttgcagatctgcgactctagaggatctgcgactctagaggatcataatcagccataccacatttgtagaggttttacttgctttaaaaaacctcccacacctccccctgaacctgaaacataaaatgaatgcaattgttgttgttaacttgtttattgcagcttataatggttacaaataaagcaatagcatcacaaatttcacaaataaagcatttttttcactgcattctagttgtggtttgtccaaactcatcaatgtatcttatcatgtctggatctgcgactctagaggatcataatcagccataccacatttgtagaggttttacttgctttaaaaaacctcccacacctccccctgaacctgaaacataaaatgaatgcaattgttgttgttaacttgtttattgcagcttataatggttacaaataaagcaatagcatcacaaatttcacaaataaagcatttttttcactgcattctagttgtggtttgtccaaactcatcaatgtatcttatcatgtctggatctgcgactctagaggatcataatcagccataccacatttgtagaggttttacttgctttaaaaaacctcccacacctccccctgaacctgaaacataaaatgaatgcaattgttgttgttaacttgtttattgcagcttataatggttacaaataaagcaatagcatcacaaatttcacaaataaagcatttttttcactgcattctagttgtggtttgtccaaactcatcaatgtatcttatcatgtctggatccccatcaagctgatccggaacccttaatataacttcgtataatgtatgctatacgaagttattaggtccctcgacctgcagcccaagctagtgcccgggtaggtccctcgacctgcagcccaagctagatcgaattcggccggccttcgaacacgtgccaccatggactataaggaccacgacggagactacaaggatcatgatattgattacaaagacgatgacgataagatggacaagcccaagaaaaagcggaaagtgaagtacagcatcggcctggacatcggcaccaactctgtgggctgggccgtgatcaccgacgagtacaaggtgcccagcaagaaattcaaggtgctgggcaacaccgacaggcacagcatcaagaagaacctgatcggcgccctgctgttcgacagcggcgaaacagccgaggccaccagactgaagagaaccgccagaagaagatacaccaggcggaagaacaggatctgctatctgcaagagatcttcagcaacgagatggccaaggtggacgacagcttcttccacagactggaagagtccttcctggtggaagaggacaagaagcacgagagacaccccatcttcggcaacatcgtggacgaggtggcctaccacgagaagtaccccaccatctaccacctgagaaagaaactggtggacagcaccgacaaggccgacctgagactgatctacctggccctggcccacatgatcaagttcagaggccacttcctgatcgagggcgacctgaaccccgacaacagcgacgtggacaagctgttcatccagctggtgcagacctacaaccagctgttcgaggaaaaccccatcaacgccagcggcgtggacgccaaggctatcctgtctgccagactgagcaagagcagaaggctggaaaatctgatcgcccagctgcccggcgagaagaagaacggcctgttcggcaacctgattgccctgagcctgggcctgacccccaacttcaagagcaacttcgacctggccgaggatgccaaactgcagctgagcaaggacacctacgacgacgacctggacaacctgctggcccagatcggcgaccagtacgccgacctgttcctggccgccaagaacctgtctgacgccatcctgctgagcgacatcctgagagtgaacaccgagatcaccaaggcccccctgagcgcctctatgatcaagagatacgacgagcaccaccaggacctgaccctgctgaaagctctcgtgcggcagcagctgcctgagaagtacaaagaaatcttcttcgaccagagcaagaacggctacgccggctacatcgatggcggcgctagccaggaagagttctacaagttcatcaagcccatcctggaaaagatggacggcaccgaggaactgctcgtgaagctgaacagagaggacctgctgagaaagcagagaaccttcgacaacggcagcatcccccaccagatccacctgggagagctgcacgctatcctgagaaggcaggaagatttttacccattcctgaaggacaaccgggaaaagatcgagaagatcctgaccttcaggatcccctactacgtgggccccctggccagaggcaacagcagattcgcctggatgaccagaaagagcgaggaaaccatcaccccctggaacttcgaggaagtggtggacaagggcgccagcgcccagagcttcatcgagagaatgacaaacttcgataagaacctgcccaacgagaaggtgctgcccaagcacagcctgctgtacgagtacttcaccgtgtacaacgagctgaccaaagtgaaatacgtgaccgagggaatgagaaagcccgccttcctgagcggcgagcagaaaaaggccatcgtggacctgctgttcaagaccaacagaaaagtgaccgtgaagcagctgaaagaggactacttcaagaaaatcgagtgcttcgactccgtggaaatctccggcgtggaagatagattcaacgcctccctgggcacataccacgatctgctgaaaattatcaaggacaaggacttcctggataacgaagagaacgaggacattctggaagatatcgtgctgaccctgacactgtttgaggaccgcgagatgatcgaggaaaggctgaaaacctacgctcacctgttcgacgacaaagtgatgaagcagctgaagagaaggcggtacaccggctggggcaggctgagcagaaagctgatcaacggcatcagagacaagcagagcggcaagacaatcctggatttcctgaagtccgacggcttcgccaaccggaacttcatgcagctgatccacgacgacagcctgacattcaaagaggacatccagaaagcccaggtgtccggccagggcgactctctgcacgagcatatcgctaacctggccggcagccccgctatcaagaagggcatcctgcagacagtgaaggtggtggacgagctcgtgaaagtgatgggcagacacaagcccgagaacatcgtgatcgagatggctagagagaaccagaccacccagaagggacagaagaactcccgcgagaggatgaagagaatcgaagagggcatcaaagagctgggcagccagatcctgaaagaacaccccgtggaaaacacccagctgcagaacgagaagctgtacctgtactacctgcagaatggccgggatatgtacgtggaccaggaactggacatcaacagactgtccgactacgatgtggaccatatcgtgcctcagagctttctgaaggacgactccatcgataacaaagtgctgactcggagcgacaagaacagaggcaagagcgacaacgtgccctccgaagaggtcgtgaagaagatgaagaactactggcgacagctgctgaacgccaagctgattacccagaggaagttcgataacctgaccaaggccgagagaggcggcctgagcgagctggataaggccggcttcatcaagaggcagctggtggaaaccagacagatcacaaagcacgtggcacagatcctggactcccggatgaacactaagtacgacgaaaacgataagctgatccgggaagtgaaagtgatcaccctgaagtccaagctggtgtccgatttccggaaggatttccagttttacaaagtgcgcgagatcaacaactaccaccacgcccacgacgcctacctgaacgccgtcgtgggaaccgccctgatcaaaaagtaccctaagctggaaagcgagttcgtgtacggcgactacaaggtgtacgacgtgcggaagatgatcgccaagagcgagcaggaaatcggcaaggctaccgccaagtacttcttctacagcaacatcatgaactttttcaagaccgaaatcaccctggccaacggcgagatcagaaagcgccctctgatcgagacaaacggcgaaaccggggagatcgtgtgggataagggcagagacttcgccacagtgcgaaaggtgctgagcatgccccaagtgaatatcgtgaaaaagaccgaggtgcagacaggcggcttcagcaaagagtctatcctgcccaagaggaacagcgacaagctgatcgccagaaagaaggactgggaccccaagaagtacggcggcttcgacagccctaccgtggcctactctgtgctggtggtggctaaggtggaaaagggcaagtccaagaaactgaagagtgtgaaagagctgctggggatcaccatcatggaaagaagcagctttgagaagaaccctatcgactttctggaagccaagggctacaaagaagtgaaaaaggacctgatcatcaagctgcctaagtactccctgttcgagctggaaaacggcagaaagagaatgctggcctctgccggcgaactgcagaagggaaacgagctggccctgcctagcaaatatgtgaacttcctgtacctggcctcccactatgagaagctgaagggcagccctgaggacaacgaacagaaacagctgtttgtggaacagcataagcactacctggacgagatcatcgagcagatcagcgagttctccaagagagtgatcctggccgacgccaatctggacaaggtgctgtctgcctacaacaagcacagggacaagcctatcagagagcaggccgagaatatcatccacctgttcaccctgacaaacctgggcgctcctgccgccttcaagtactttgacaccaccatcgaccggaagaggtacaccagcaccaaagaggtgctggacgccaccctgatccaccagagcatcaccggcctgtacgagacaagaatcgacctgtctcagctgggaggcgacaagagacctgccgccactaagaaggccggacaggccaaaaagaagaagtgataaatgcatggccggccctgcaggaattcgatatcaagcttatcgataatcaacctctggattacaaaatttgtgaaagattgactggtattcttaactatgttgctccttttacgctatgtggatacgctgctttaatgcctttgtatcatgctattgcttcccgtatggctttcattttctcctccttgtataaatcctggttgctgtctctttatgaggagttgtggcccgttgtcaggcaacgtggcgtggtgtgcactgtgtttgctgacgcaacccccactggttggggcattgccaccacctgtcagctcctttccgggactttcgctttccccctccctattgccacggcggaactcatcgccgcctgccttgcccgctgctggacaggggctcggctgttgggcactgacaattccgtggtgttgtcggggaaatcatcgtcctttccttggctgctcgcctgtgttgccacctggattctgcgcgggacgtccttctgctacgtcccttcggccctcaatccagcggaccttccttcccgcggcctgctgccggctctgcggcctcttccgcgtcttcgccttcgccctcagacgagtcggatctccctttgggccgcctccccgcatcgataccgtcgacctcgacctcgactgtgccttctagttgccagccatctgttgtttgcccctcccccgtgccttccttgaccctggaaggtgccactcccactgtcctttcctaataaaatgaggaaattgcatcgcattgtctgagtaggtgtcattctattctggggggtggggtggggcaggacagcaagggggaggattgggaagacaatggcaggcatgctggggaactagtggtgccagggcgtgcccttgggctccccgggcgcggcggccatcgctcgagtaaaattggagggacaagacttcccacagattttcggttttgtcgggaagttttttaataggggcaaataaggaaaatgggaggataggtagtcatctggggttttatgcagcaaaactacaggttattattgcttgtgatccgc

SEQ ID NO: 21 - DNA, 7456 bp, Artificial Sequence
  Synthetic
  misc_feature (1)..(170): Mouse Rosa26 Upstream
  misc_feature (205)..(1923): CAGG Promoter
  misc_feature (2006)..(2039): LoxP
  misc_feature (2134)..(2143): Kozak
  misc_feature (2143)..(2208): 3xFLAG
  misc_feature (2209)..(6381): Cas9
  misc_feature (2218)..(2238): Monopartite NLS
  misc_feature (6334)..(6381): Bipartite NLS
  misc_feature (6428)..(7024): WPRE
  misc_feature (7032)..(7247): bGH PolyA
  misc_feature (7307)..(7456): Mouse Rosa26 Downstream
ctgcagtggagtaggcggggagaaggccgcacccttctccggaggggggaggggagtgttgcaatacctttctgggagttctctgctgcctcctggcttctgaggaccgccctgggcctgggagaatcccttccccctcttccctcgtgatctgcaactccagtctttctccttaattaaacgcgtctggcctcgcgagtgtgtactagttattaatagtaatcaattacggggtcattagttcatagcccatatatggagttccgcgttacataacttacggtaaatggcccgcctggctgaccgcccaacgacccccgcccattgacgtcaataatgacgtatgttcccatagtaacgccaatagggactttccattgacgtcaatgggtggagtatttacggtaaactgcccacttggcagtacatcaagtgtatcatatgccaagtacgccccctattgacgtcaatgacggtaaatggcccgcctggcattatgcccagtacatgaccttatgggactttcctacttggcagtacatctacgtattagtcatcgctattaccatggtcgaggtgagccccacgttctgcttcactctccccatctcccccccctccccacccccaattttgtatttatttattttttaattattttgtgcagcgatgggggcggggggggggggggggcgcgcgccaggcggggcggggcggggcgaggggcggggcggggcgaggcggagaggtgcggcggcagccaatcagagcggcgcgctccgaaagtttccttttatggcgaggcggcggcggcggcggccctataaaaagcgaagcgcgcggcgggcggggagtcgctgcgacgctgccttcgccccgtgccccgctccgccgccgcctcgcgccgcccgccccggctctgactgaccgcgttactcccacaggtgagcgggcgggacggcccttctcctccgggctgtaattagcgcttggtttaatgacggcttgtttcttttctgtggctgcgtgaaagccttgaggggctccgggagggccctttgtgcggggggagcggctcggggggtgcgtgcgtgtgtgtgtgcgtggggagcgccgcgtgcggctccgcgctgcccggcggctgtgagcgctgcgggcgcggcgcggggctttgtgcgctccgcagtgtgcgcgaggggagcgcggccgggggcggtgccccgcggtgcggggggggctgcgaggggaacaaaggctgcgtgcggggtgtgtgcgtgggggggtgagcagggggtgtgggcgcgtcggtcgggctgcaaccccccctgcacccccctccccgagttgctgagcacggcccggcttcgggtgcggggctccgtacggggcgtggcgcggggctcgccgtgccgggcggggggtggcggcaggtgggggtgccgggcggggcggggccgcctcgggccggggagggctcgggggaggggcgcggcggcccccggagcgccggcggctgtcgaggcgcggcgagccgcagccattgccttttatggtaatcgtgcgagagggcgcagggacttcctttgtcccaaatctgtgcggagccgaaatctgggaggcgccgccgcaccccctctagcgggcgcggggcgaagcggtgcggcgccggcaggaaggaaatgggcggggagggccttcgtgcgtcgccgcgccgccgtccccttctccctctccagcctcggggctgtccgcggggggacggctgccttcgggggggacggggcagggcggggttcggcttctggcgtgtgaccggcggctctagagcctctgctaaccatgttcatgccttcttctttttcctacagctcctgggcaacgtgctggttattgtgctgtctcatcattttggcaaagaattcgctaggagaattgatttgataccgcgggccctaagtcgacatttaaatcatttaaatccactagtggatccggaacccttaatataacttcgtataatgtatgctatacgaagttattaggtccctcgacctgcagcccaagctagtgcccgggtaggtccctcgacctgcagcccaagctagatcgaattcggccggccttcgaacacgtgccaccatggactataaggaccacgacggagactacaaggatcatgatattgattacaaagacgatgacgataagatggacaagcccaagaaaaagcggaaagtgaagtacagcatcggcctggacatcggcaccaactctgtgggctgggccgtgatcaccgacgagtacaaggtgcccagcaagaaattcaaggtgctgggcaacaccgacaggcacagcatcaagaagaacctgatcggcgccctgctgttcgacagcggcgaaacagccgaggccaccagactgaagagaaccgccagaagaagatacaccaggcggaagaacaggatctgctatctgcaagagatcttcagcaacgagatggccaaggtggacgacagcttcttccacagactggaagagtccttcctggtggaagaggacaagaagcacgagagacaccccatcttcggcaacatcgtggacgaggtggcctaccacgagaagtaccccaccatctaccacctgagaaagaaactggtggacagcaccgacaaggccgacctgagactgatctacctggccctggcccacatgatcaagttcagaggccacttcctgatcgagggcgacctgaaccccgacaacagcgacgtggacaagctgttcatccagctggtgcagacctacaaccagctgttcgaggaaaaccccatcaacgccagcggcgtggacgccaaggctatcctgtctgccagactgagcaagagcagaaggctggaaaatctgatcgcccagctgcccggcgagaagaagaacggcctgttcggcaacctgattgccctgagcctgggcctgacccccaacttcaagagcaacttcgacctggccgaggatgccaaactgcagctgagcaaggacacctacgacgacgacctggacaacctgctggcccagatcggcgaccagtacgccgacctgttcctggccgccaagaacctgtctgacgccatcctgctgagcgacatcctgagagtgaacaccgagatcaccaaggcccccctgagcgcctctatgatcaagagatacgacgagcaccaccaggacctgaccctgctgaaagctctcgtgcggcagcagctgcctgagaagtacaaagaaatcttcttcgaccagagcaagaacggctacgccggctacatcgatggcggcgctagccaggaagagttctacaagttcatcaagcccatcctggaaaagatggacggcaccgaggaactgctcgtgaagctgaacagagaggacctgctgagaaagcagagaaccttcgacaacggcagcatcccccaccagatccacctgggagagctgcacgctatcctgagaaggcaggaagatttttacccattcctgaaggacaaccgggaaaagatcgagaagatcctgaccttcaggatcccctactacgtgggccccctggccagaggcaacagcagattcgcctggatgaccagaaagagcgaggaaaccatcaccccctggaacttcgaggaagtggtggacaagggcgccagcgcccagagcttcatcgagagaatgacaaacttcgataagaacctgcccaacgagaaggtgctgcccaagcacagcctgctgtacgagtacttcaccgtgtacaacgagctgaccaaagtgaaatacgtgaccgagggaatgagaaagcccgccttcctgagcggcgagcagaaaaaggccatcgtggacctgctgttcaagaccaacagaaaagtgaccgtgaagcagctgaaagaggactacttcaagaaaatcgagtgcttcgactccgtggaaatctccggcgtggaagatagattcaacgcctccctgggcacataccacgatctgctgaaaattatcaaggacaaggacttcctggataacgaagagaacgaggacattctggaagatatcgtgctgaccctgacactgtttgaggaccgcgagatgatcgaggaaaggctgaaaacctacgctcacctgttcgacgacaaagtgatgaagcagctgaagagaaggcggtacaccggctggggcaggctgagcagaaagctgatcaacggcatcagagacaagcagagcggcaagacaatcctggatttcctgaagtccgacggcttcgccaaccggaacttcatgcagctgatccacgacgacagcctgacattcaaagaggacatccagaaagcccaggtgtccggccagggcgactctctgcacgagcatatcgctaacctggccggcagccccgctatcaagaagggcatcctgcagacagtgaaggtggtggacgagctcgtgaaagtgatgggcagacacaagcccgagaacatcgtgatcgagatggctagagagaaccagaccacccagaagggacagaagaactcccgcgagaggatgaagagaatcgaagagggcatcaaagagctgggcagccagatcctgaaagaacaccccgtggaaaacacccagctgcagaacgagaagctgtacctgtactacctgcagaatggccgggatatgtacgtggaccaggaactggacatcaacagactgtccgactacgatgtggaccatatcgtgcctcagagctttctgaaggacgactccatcgataacaaagtgctgactcggagcgacaagaacagaggcaagagcgacaacgtgccctccgaagaggtcgtgaagaagatgaagaactactggcgacagctgctgaacgccaagctgattacccagaggaagttcgataacctgaccaaggccgagagaggcggcctgagcgagctggataaggccggcttcatcaagaggcagctggtggaaaccagacagatcacaaagcacgtggcacagatcctggactcccggatgaacactaagtacgacgaaaacgataagctgatccgggaagtgaaagtgatcaccctgaagtccaagctggtgtccgatttccggaaggatttccagttttacaaagtgcgcgagatcaacaactaccaccacgcccacgacgcctacctgaacgccgtcgtgggaaccgccctgatcaaaaagtaccctaagctggaaagcgagttcgtgtacggcgactacaaggtgtacgacgtgcggaagatgatcgccaagagcgagcaggaaatcggcaaggctaccgccaagtacttcttctacagcaacatcatgaactttttcaagaccgaaatcaccctggccaacggcgagatcagaaagcgccctctgatcgagacaaacggcgaaaccggggagatcgtgtgggataagggcagagacttcgccacagtgcgaaaggtgctgagcatgccccaagtgaatatcgtgaaaaagaccgaggtgcagacaggcggcttcagcaaagagtctatcctgcccaagaggaacagcgacaagctgatcgccagaaagaaggactgggaccccaagaagtacggcggcttcgacagccctaccgtggcctactctgtgctggtggtggctaaggtggaaaagggcaagtccaagaaactgaagagtgtgaaagagctgctggggatcaccatcatggaaagaagcagctttgagaagaaccctatcgactttctggaagccaagggctacaaagaagtgaaaaaggacctgatcatcaagctgcctaagtactccctgttcgagctggaaaacggcagaaagagaatgctggcctctgccggcgaactgcagaagggaaacgagctggccctgcctagcaaatatgtgaacttcctgtacctggcctcccactatgagaagctgaagggcagccctgaggacaacgaacagaaacagctgtttgtggaacagcataagcactacctggacgagatcatcgagcagatcagcgagttctccaagagagtgatcctggccgacgccaatctggacaaggtgctgtctgcctacaacaagcacagggacaagcctatcagagagcaggccgagaatatcatccacctgttcaccctgacaaacctgggcgctcctgccgccttcaagtactttgacaccaccatcgaccggaagaggtacaccagcaccaaagaggtgctggacgccaccctgatccaccagagcatcaccggcctgtacgagacaagaatcgacctgtctcagctgggaggcgacaagagacctgccgccactaagaaggccggacaggccaaaaagaagaagtgataaatgcatggccggccctgcaggaattcgatatcaagcttatcgataatcaacctctggattacaaaatttgtgaaagattgactggtattcttaactatgttgctccttttacgctatgtggatacgctgctttaatgcctttgtatcatgctattgcttcccgtatggctttcattttctcctccttgtataaatcctggttgctgtctctttatgaggagttgtggcccgttgtcaggcaacgtggcgtggtgtgcactgtgtttgctgacgcaacccccactggttggggcattgccaccacctgtcagctcctttccgggactttcgctttccccctccctattgccacggcggaactcatcgccgcctgccttgcccgctgctggacaggggctcggctgttgggcactgacaattccgtggtgttgtcggggaaatcatcgtcctttccttggctgctcgcctgtgttgccacctggattctgcgcgggacgtccttctgctacgtcccttcggccctcaatccagcggaccttccttcccgcggcctgctgccggctctgcggcctcttccgcgtcttcgccttcgccctcagacgagtcggatctccctttgggccgcctccccgcatcgataccgtcgacctcgacctcgactgtgccttctagttgccagccatctgttgtttgcccctcccccgtgccttccttgaccctggaaggtgccactcccactgtcctttcctaataaaatgaggaaattgcatcgcattgtctgagtaggtgtcattctattctggggggtggggtggggcaggacagcaagggggaggattgggaagacaatggcaggcatgctggggaactagtggtgccagggcgtgcccttgggctccccgggcgcggcggccatcgctcgagtaaaattggagggacaagacttcccacagattttcggttttgtcgggaagttttttaataggggcaaataaggaaaatgggaggataggtagtcatctggggttttatgcagcaaaactacaggttattattgcttgtgatccgc

SEQ ID NO: 22 - protein, 1413 aa, Artificial Sequence
  Synthetic
  MISC_FEATURE (1)..(22): 3xFLAG
  MISC_FEATURE (23)..(1413): Cas9
DYKDHDGDYKDHDIDYKDDDDKMDKPKKKRKVKYSIGLDIGTNSVGWAVITDEYKVPSKKFKVLGNTDRHSIKKNLIGALLFDSGETAEATRLKRTARRRYTRRKNRICYLQEIFSNEMAKVDDSFFHRLEESFLVEEDKKHERHPIFGNIVDEVAYHEKYPTIYHLRKKLVDSTDKADLRLIYLALAHMIKFRGHFLIEGDLNPDNSDVDKLFIQLVQTYNQLFEENPINASGVDAKAILSARLSKSRRLENLIAQLPGEKKNGLFGNLIALSLGLTPNFKSNFDLAEDAKLQLSKDTYDDDLDNLLAQIGDQYADLFLAAKNLSDAILLSDILRVNTEITKAPLSASMIKRYDEHHQDLTLLKALVRQQLPEKYKEIFFDQSKNGYAGYIDGGASQEEFYKFIKPILEKMDGTEELLVKLNREDLLRKQRTFDNGSIPHQIHLGELHAILRRQEDFYPFLKDNREKIEKILTFRIPYYVGPLARGNSRFAWMTRKSEETITPWNFEEVVDKGASAQSFIERMTNFDKNLPNEKVLPKHSLLYEYFTVYNELTKVKYVTEGMRKPAFLSGEQKKAIVDLLFKTNRKVTVKQLKEDYFKKIECFDSVEISGVEDRFNASLGTYHDLLKIIKDKDFLDNEENEDILEDIVLTLTLFEDREMIEERLKTYAHLFDDKVMKQLKRRRYTGWGRLSRKLINGIRDKQSGKTILDFLKSDGFANRNFMQLIHDDSLTFKEDIQKAQVSGQGDSLHEHIANLAGSPAIKKGILQTVKVVDELVKVMGRHKPENIVIEMARENQTTQKGQKNSRERMKRIEEGIKELGSQILKEHPVENTQLQNEKLYLYYLQNGRDMYVDQELDINRLSDYDVDHIVPQSFLKDDSIDNKVLTRSDKNRGKSDNVPSEEVVKKMKNYWRQLLNAKLITQRKFDNLTKAERGGLSELDKAGFIKRQLVETRQITKHVAQILDSRMNTKYDENDKLIREVKVITLKSKLVSDFRKDFQFYKVREINNYHHAHDAYLNAVVGTALIKKYPKLESEFVYGDYKVYDVRKMIAKSEQEIGKATAKYFFYSNIMNFFKTEITLANGEIRKRPLIETNGETGEIVWDKGRDFATVRKVLSMPQVNIVKKTEVQTGGFSKESILPKRNSDKLIARKKDWDPKKYGGFDSPTVAYSVLVVAKVEKGKSKKLKSVKELLGITIMERSSFEKNPIDFLEAKGYKEVKKDLIIKLPKYSLFELENGRKRMLASAGELQKGNELALPSKYVNFLYLASHYEKLKGSPEDNEQKQLFVEQHKHYLDEIIEQISEFSKRVILADANLDKVLSAYNKHRDKPIREQAENIIHLFTLTNLGAPAAFKYFDTTIDRKRYTSTKEVLDATLIHQSITGLYETRIDLSQLGGDKRPAATKKAGQAKKKK

SEQ ID NO: 23 - protein, 22 aa, Artificial Sequence
  Synthetic
DYKDHDGDYKDHDIDYKDDDDK

SEQ ID NO: 24 - protein, 238 aa, Artificial Sequence
  Synthetic
VSKGEELFTGVVPILVELDGDVNGHKFSVSGEGEGDATYGKLTLKFICTTGKLPVPWPTLVTTLTYGVQCFSRYPDHMKQHDFFKSAMPEGYVQERTIFFKDDGNYKTRAEVKFEGDTLVNRIELKGIDFKEDGNILGHKLEYNYNSHNVYIMADKQKNGIKVNFKIRHNIEDGSVQLADHYQQNTPIGDGPVLLPDNHYLSTQSALSKDPNEKRDHMVLLEFVTAAGITLGMDELYK

SEQ ID NO: 25 - RNA, 16 nt, Artificial Sequence
  Synthetic
guuuuagagcuaugcu

SEQ ID NO: 26 - RNA, 67 nt, Artificial Sequence
  Synthetic
agcauagcaaguuaaaauaaggcuaguccguuaucaacuugaaaaaguggcaccgagucggugcuuu

SEQ ID NO: 27 - RNA, 77 nt, Artificial Sequence
  Synthetic
guuuuagagcuagaaauagcaaguuaaaauaaggcuaguccguuaucaacuugaaaaaguggcaccgagucggugcu

SEQ ID NO: 28 - DNA, 4953 bp, Artificial Sequence
  Synthetic
  misc_feature (1)..(4173): Cas9
  misc_feature (4174)..(4239): P2A
  misc_feature (4240)..(4953): eGFP
atggacaagcccaagaaaaagcggaaagtgaagtacagcatcggcctggacatcggcaccaactctgtgggctgggccgtgatcaccgacgagtacaaggtgcccagcaagaaattcaaggtgctgggcaacaccgacaggcacagcatcaagaagaacctgatcggcgccctgctgttcgacagcggcgaaacagccgaggccaccagactgaagagaaccgccagaagaagatacaccaggcggaagaacaggatctgctatctgcaagagatcttcagcaacgagatggccaaggtggacgacagcttcttccacagactggaagagtccttcctggtggaagaggacaagaagcacgagagacaccccatcttcggcaacatcgtggacgaggtggcctaccacgagaagtaccccaccatctaccacctgagaaagaaactggtggacagcaccgacaaggccgacctgagactgatctacctggccctggcccacatgatcaagttcagaggccacttcctgatcgagggcgacctgaaccccgacaacagcgacgtggacaagctgttcatccagctggtgcagacctacaaccagctgttcgaggaaaaccccatcaacgccagcggcgtggacgccaaggctatcctgtctgccagactgagcaagagcagaaggctggaaaatctgatcgcccagctgcccggcgagaagaagaacggcctgttcggcaacctgattgccctgagcctgggcctgacccccaacttcaagagcaacttcgacctggccgaggatgccaaactgcagctgagcaaggacacctacgacgacgacctggacaacctgctggcccagatcggcgaccagtacgccgacctgttcctggccgccaagaacctgtctgacgccatcctgctgagcgacatcctgagagtgaacaccgagatcaccaaggcccccctgagcgcctctatgatcaagagatacgacgagcaccaccaggacctgaccctgctgaaagctctcgtgcggcagcagctgcctgagaagtacaaagaaatcttcttcgaccagagcaagaacggctacgccggctacatcgatggcggcgctagccaggaagagttctacaagttcatcaagcccatcctggaaaagatggacggcaccgaggaactgctcgtgaagctgaacagagaggacctgctgagaaagcagagaaccttcgacaacggcagcatcccccaccagatccacctgggagagctgcacgctatcctgagaaggcaggaagatttttacccattcctgaaggacaaccgggaaaagatcgagaagatcctgaccttcaggatcccctactacgtgggccccctggccagaggcaacagcagattcgcctggatgaccagaaagagcgaggaaaccatcaccccctggaacttcgaggaagtggtggacaagggcgccagcgcccagagcttcatcgagagaatgacaaacttcgataagaacctgcccaacgagaaggtgctgcccaagcacagcctgctgtacgagtacttcaccgtgtacaacgagctgaccaaagtgaaatacgtgaccgagggaatgagaaagcccgccttcctgagcggcgagcagaaaaaggccatcgtggacctgctgttcaagaccaacagaaaagtgaccgtgaagcagctgaaagaggactacttcaagaaaatcgagtgcttcgactccgtggaaatctccggcgtggaagatagattcaacgcctccctgggcacataccacgatctgctgaaaattatcaaggacaaggacttcctggataacgaagagaacgaggacattctggaagatatcgtgctgaccctgacactgtttgaggaccgcgagatgatcgaggaaaggctgaaaacctacgctcacctgttcgacgacaaagtgatgaagcagctgaagagaaggcggtacaccggctggggcaggctgagcagaaagctgatcaacggcatcagagacaagcagagcggcaagacaatcctggatttcctgaagtccgacggcttcgccaaccggaacttcatgcagctgatccacgacgacagcctgacattcaaagaggacatccagaaagcccaggtgtccggccagggcgactctctgcacgagcatatcgctaacctggccggcagccccgctatcaagaagggcatcctgcagacagtgaaggtggtggacgagctcgtgaaagtgatgggcagacacaagcccgagaacatcgtgatcgagatggctagagagaaccagaccacccagaagggacagaagaactcccgcgagaggatgaagagaatcgaagagggcatcaaagagctgggcagccagatcctgaaagaacaccccgtggaaaacacccagctgcagaacgagaagctgtacctgtactacctgcagaatggccgggatatgtacgtggaccaggaactggacatcaacagactgtccgactacgatgtggaccatatcgtgcctcagagctttctgaaggacgactccatcgataacaaagtgctgactcggagcgacaagaacagaggcaagagcgacaacgtgccctccgaagaggtcgtgaagaagatgaagaactactggcgacagctgctgaacgccaagctgattacccagaggaagttcgataacctgaccaaggccgagagaggcggcctgagcgagctggataaggccggcttcatcaagaggcagctggtggaaaccagacagatcacaaagcacgtggcacagatcctggactcccggatgaacactaagtacgacgaaaacgataagctgatccgggaagtgaaagtgatcaccctgaagtccaagctggtgtccgatttccggaaggatttccagttttacaaagtgcgcgagatcaacaactaccaccacgcccacgacgcctacctgaacgccgtcgtgggaaccgccctgatcaaaaagtaccctaagctggaaagcgagttcgtgtacggcgactacaaggtgtacgacgtgcggaagatgatcgccaagagcgagcaggaaatcggcaaggctaccgccaagtacttcttctacagcaacatcatgaactttttcaagaccgaaatcaccctggccaacggcgagatcagaaagcgccctctgatcgagacaaacggcgaaaccggggagatcgtgtgggataagggcagagacttcgccacagtgcgaaaggtgctgagcatgccccaagtgaatatcgtgaaaaagaccgaggtgcagacaggcggcttcagcaaagagtctatcctgcccaagaggaacagcgacaagctgatcgccagaaagaaggactgggaccccaagaagtacggcggcttcgacagccctaccgtggcctactctgtgctggtggtggctaaggtggaaaagggcaagtccaagaaactgaagagtgtgaaagagctgctggggatcaccatcatggaaagaagcagctttgagaagaaccctatcgactttctggaagccaagggctacaaagaagtgaaaaaggacctgatcatcaagctgcctaagtactccctgttcgagctggaaaacggcagaaagagaatgctggcctctgccggcgaactgcagaagggaaacgagctggccctgcctagcaaatatgtgaacttcctgtacctggcctcccactatgagaagctgaagggcagccctgaggacaacgaacagaaacagctgtttgtggaacagcataagcactacctggacgagatcatcgagcagatcagcgagttctccaagagagtgatcctggccgacgccaatctggacaaggtgctgtctgcctacaacaagcacagggacaagcctatcagagagcaggccgagaatatcatccacctgttcaccctgacaaacctgggcgctcctgccgccttcaagtactttgacaccaccatcgaccggaagaggtacaccagcaccaaagaggtgctggacgccaccctgatccaccagagcatcaccggcctgtacgagacaagaatcgacctgtctcagctgggaggcgacaagagacctgccgccactaagaaggccggacaggccaaaaagaagaagggaagcggagccactaacttctccctgttgaaacaagcaggggatgtcgaagagaatcccgggccagtgagcaagggcgaggagctgttcaccggggtggtgcccatcctggtcgagctggacggcgacgtaaacggccacaagttcagcgtgtccggcgagggcgagggcgatgccacctacggcaagctgaccctgaagttcatctgcaccaccggcaagctgcccgtgccctggcccaccctcgtgaccaccctgacctacggcgtgcagtgcttcagccgctaccccgaccacatgaagcagcacgacttcttcaagtccgccatgcccgaaggctacgtccaggagcgcaccatcttcttcaaggacgacggcaactacaagacccgcgccgaggtgaagttcgagggcgacaccctggtgaaccgcatcgagctgaagggcatcgacttcaaggaggacggcaacatcctggggcacaagctggagtacaactacaacagccacaacgtctatatcatggccgacaagcagaagaacggcatcaaggtgaacttcaagatccgccacaacatcgaggacggcagcgtgcagctcgccgaccactaccagcagaacacccccatcggcgacggccccgtgctgctgcccgacaaccactacctgagcacccagtccgccctgagcaaagaccccaacgagaagcgcgatcacatggtcctgctggagttcgtgaccgccgccgggatcactctcggcatggacgagctgtacaag

SEQ ID NO: 29 - DNA, 5019 bp, Artificial Sequence
  Synthetic
  misc_feature (1)..(66): 3xFLAG
  misc_feature (67)..(4239): Cas9
  misc_feature (4240)..(4305): P2A
  misc_feature (4306)..(5019): eGFP
gactataaggaccacgacggagactacaaggatcatgatattgattacaaagacgatgacgataagatggacaagcccaagaaaaagcggaaagtgaagtacagcatcggcctggacatcggcaccaactctgtgggctgggccgtgatcaccgacgagtacaaggtgcccagcaagaaattcaaggtgctgggcaacaccgacaggcacagcatcaagaagaacctgatcggcgccctgctgttcgacagcggcgaaacagccgaggccaccagactgaagagaaccgccagaagaagatacaccaggcggaagaacaggatctgctatctgcaagagatcttcagcaacgagatggccaaggtggacgacagcttcttccacagactggaagagtccttcctggtggaagaggacaagaagcacgagagacaccccatcttcggcaacatcgtggacgaggtggcctaccacgagaagtaccccaccatctaccacctgagaaagaaactggtggacagcaccgacaaggccgacctgagactgatctacctggccctggcccacatgatcaagttcagaggccacttcctgatcgagggcgacctgaaccccgacaacagcgacgtggacaagctgttcatccagctggtgcagacctacaaccagctgttcgaggaaaaccccatcaacgccagcggcgtggacgccaaggctatcctgtctgccagactgagcaagagcagaaggctggaaaatctgatcgcccagctgcccggcgagaagaagaacggcctgttcggcaacctgattgccctgagcctgggcctgacccccaacttcaagagcaacttcgacctggccgaggatgccaaactgcagctgagcaaggacacctacgacgacgacctggacaacctgctggcccagatcggcgaccagtacgccgacctgttcctggccgccaagaacctgtctgacgccatcctgctgagcgacatcctgagagtgaacaccgagatcaccaaggcccccctgagcgcctctatgatcaagagatacgacgagcaccaccaggacctgaccctgctgaaagctctcgtgcggcagcagctgcctgagaagtacaaagaaatcttcttcgaccagagcaagaacggctacgccggctacatcgatggcggcgctagccaggaagagttctacaagttcatcaagcccatcctggaaaagatggacggcaccgaggaactgctcgtgaagctgaacagagaggacctgctgagaaagcagagaaccttcgacaacggcagcatcccccaccagatccacctgggagagctgcacgctatcctgagaaggcaggaagatttttacccattcctgaaggacaaccgggaaaagatcgagaagatcctgaccttcaggatcccctactacgtgggccccctggccagaggcaacagcagattcgcctggatgaccagaaagagcgaggaaaccatcaccccctggaacttcgaggaagtggtggacaagggcgccagcgcccagagcttcatcgagagaatgacaaacttcgataagaacctgcccaacgagaaggtgctgcccaagcacagcctgctgtacgagtacttcaccgtgtacaacgagctgaccaaagtgaaatacgtgaccgagggaatgagaaagcccgccttcctgagcggcgagcagaaaaaggccatcgtggacctgctgttcaagaccaacagaaaagtgaccgtgaagcagctgaaagaggactacttcaagaaaatcgagtgcttcgactccgtggaaatctccggcgtggaagatagattcaacgcctccctgggcacataccacgatctgctgaaaattatcaaggacaaggacttcctggataacgaagagaacgaggacattctggaagatatcgtgctgaccctgacactgtttgaggaccgcgagatgatcgaggaaaggctgaaaacctacgctcacctgttcgacgacaaagtgatgaagcagctgaagagaaggcggtacaccggctggggcaggctgagcagaaagctgatcaacggcatcagagacaagcagagcggcaagacaatcctggatttcctgaagtccgacggcttcgccaaccggaacttcatgcagctgatccacgacgacagcctgacattcaaagaggacatccagaaagcccaggtgtccggccagggcgactctctgcacgagcatatcgctaacctggccggcagccccgctatcaagaagggcatcctgcagacagtgaaggtggtggacgagctcgtgaaagtgatgggcagacacaagcccgagaacatcgtgatcgagatggctagagagaaccagaccacccagaagggacagaagaactcccgcgagaggatgaagagaatcgaagagggcatcaaagagctgggcagccagatcctgaaagaacaccccgtggaaaacacccagctgcagaacgagaagctgtacctgtactacctgcagaatggccgggatatgtacgtggaccaggaactggacatcaacagactgtccgactacgatgtggaccatatcgtgcctcagagctttctgaaggacgactccatcgataacaaagtgctgactcggagcgacaagaacagaggcaagagcgacaacgtgccctccgaagaggtcgtgaagaagatgaagaactactggcgacagctgctgaacgccaagctgattacccagaggaagttcgataacctgaccaaggccgagagaggcggcctgagcgagctggataaggccggcttcatcaagaggcagctggtggaaaccagacagatcacaaagcacgtggcacagatcctggactcccggatgaacactaagtacgacgaaaacgataagctgatccgggaagtgaaagtgatcaccctgaagtccaagctggtgtccgatttccggaaggatttccagttttacaaagtgcgcgagatcaacaactaccaccacgcccacgacgcctacctgaacgccgtcgtgggaaccgccctgatcaaaaagtaccctaagctggaaagcgagttcgtgtacggcgactacaaggtgtacgacgtgcggaagatgatcgccaagagcgagcaggaaatcggcaaggctaccgccaagtacttcttctacagcaacatcatgaactttttcaagaccgaaatcaccctggccaacggcgagatcagaaagcgccctctgatcgagacaaacggcgaaaccggggagatcgtgtgggataagggcagagacttcgccacagtgcgaaaggtgctgagcatgccccaagtgaatatcgtgaaaaagaccgaggtgcagacaggcggcttcagcaaagagtctatcctgcccaagaggaacagcgacaagctgatcgccagaaagaaggactgggaccccaagaagtacggcggcttcgacagccctaccgtggcctactctgtgctggtggtggctaaggtggaaaagggcaagtccaagaaactgaagagtgtgaaagagctgctggggatcaccatcatggaaagaagcagctttgagaagaaccctatcgactttctggaagccaagggctacaaagaagtgaaaaaggacctgatcatcaagctgcctaagtactccctgttcgagctggaaaacggcagaaagagaatgctggcctctgccggcgaactgcagaagggaaacgagctggccctgcctagcaaatatgtgaacttcctgtacctggcctcccactatgagaagctgaagggcagccctgaggacaacgaacagaaacagctgtttgtggaacagcataagcactacctggacgagatcatcgagcagatcagcgagttctccaagagagtgatcctggccgacgccaatctggacaaggtgctgtctgcctacaacaagcacagggacaagcctatcagagagcaggccgagaatatcatccacctgttcaccctgacaaacctgggcgctcctgccgccttcaagtactttgacaccaccatcgaccggaagaggtacaccagcaccaaagaggtgctggacgccaccctgatccaccagagcatcaccggcctgtacgagacaagaatcgacctgtctcagctgggaggcgacaagagacctgccgccactaagaaggccggacaggccaaaaagaagaagggaagcggagccactaacttctccctgttgaaacaagcaggggatgtcgaagagaatcccgggccagtgagcaagggcgaggagctgttcaccggggtggtgcccatcctggtcgagctggacggcgacgtaaacggccacaagttcagcgtgtccggcgagggcgagggcgatgccacctacggcaagctgaccctgaagttcatctgcaccaccggcaagctgcccgtgccctggcccaccctcgtgaccaccctgacctacggcgtgcagtgcttcagccgctaccccgaccacatgaagcagcacgacttcttcaagtccgccatgcccgaaggctacgtccaggagcgcaccatcttcttcaaggacgacggcaactacaagacccgcgccgaggtgaagttcgagggcgacaccctggtgaaccgcatcgagctgaagggcatcgacttcaaggaggacggcaacatcctggggcacaagctggagtacaactacaacagccacaacgtctatatcatggccgacaagcagaagaacggcatcaaggtgaacttcaagatccgccacaacatcgaggacggcagcgtgcagctcgccgaccactaccagcagaacacccccatcggcgacggccccgtgctgctgcccgacaaccactacctgagcacccagtccgccctgagcaaagaccccaacgagaagcgcgatcacatggtcctgctggagttcgtgaccgccgccgggatcactctcggcatggacgagctgtacaag

SEQ ID NO: 30 - DNA, 4173 bp, Artificial Sequence
  Synthetic
atggacaagcccaagaaaaagcggaaagtgaagtacagcatcggcctggacatcggcaccaactctgtgggctgggccgtgatcaccgacgagtacaaggtgcccagcaagaaattcaaggtgctgggcaacaccgacaggcacagcatcaagaagaacctgatcggcgccctgctgttcgacagcggcgaaacagccgaggccaccagactgaagagaaccgccagaagaagatacaccaggcggaagaacaggatctgctatctgcaagagatcttcagcaacgagatggccaaggtggacgacagcttcttccacagactggaagagtccttcctggtggaagaggacaagaagcacgagagacaccccatcttcggcaacatcgtggacgaggtggcctaccacgagaagtaccccaccatctaccacctgagaaagaaactggtggacagcaccgacaaggccgacctgagactgatctacctggccctggcccacatgatcaagttcagaggccacttcctgatcgagggcgacctgaaccccgacaacagcgacgtggacaagctgttcatccagctggtgcagacctacaaccagctgttcgaggaaaaccccatcaacgccagcggcgtggacgccaaggctatcctgtctgccagactgagcaagagcagaaggctggaaaatctgatcgcccagctgcccggcgagaagaagaacggcctgttcggcaacctgattgccctgagcctgggcctgacccccaacttcaagagcaacttcgacctggccgaggatgccaaactgcagctgagcaaggacacctacgacgacgacctggacaacctgctggcccagatcggcgaccagtacgccgacctgttcctggccgccaagaacctgtctgacgccatcctgctgagcgacatcctgagagtgaacaccgagatcaccaaggcccccctgagcgcctctatgatcaagagatacgacgagcaccaccaggacctgaccctgctgaaagctctcgtgcggcagcagctgcctgagaagtacaaagaaatcttcttcgaccagagcaagaacggctacgccggctacatcgatggcggcgctagccaggaagagttctacaagttcatcaagcccatcctggaaaagatggacggcaccgaggaactgctcgtgaagctgaacagagaggacctgctgagaaagcagagaaccttcgacaacggcagcatcccccaccagatccacctgggagagctgcacgctatcctgagaaggcaggaagatttttacccattcctgaaggacaaccgggaaaagatcgagaagatcctgaccttcaggatcccctactacgtgggccccctggccagaggcaacagcagattcgcctggatgaccagaaagagcgaggaaaccatcaccccctggaacttcgaggaagtggtggacaagggcgccagcgcccagagcttcatcgagagaatgacaaacttcgataagaacctgcccaacgagaaggtgctgcccaagcacagcctgctgtacgagtacttcaccgtgtacaacgagctgaccaaagtgaaatacgtgaccgagggaatgagaaagcccgccttcctgagcggcgagcagaaaaaggccatcgtggacctgctgttcaagaccaacagaaaagtgaccgtgaagcagctgaaagaggactacttcaagaaaatcgagtgcttcgactccgtggaaatctccggcgtggaagatagattcaacgcctccctgggcacataccacgatctgctgaaaattatcaaggacaaggacttcctggataacgaagagaacgaggacattctggaagatatcgtgctgaccctgacactgtttgaggaccgcgagatgatcgaggaaaggctgaaaacctacgctcacctgttcgacgacaaagtgatgaagcagctgaagagaaggcggtacaccggctggggcaggctgagcagaaagctgatcaacggcatcagagacaagcagagcggcaagacaatcctggatttcctgaagtccgacggcttcgccaaccggaacttcatgcagctgatccacgacgacagcctgacattcaaagaggacatccagaaagcccaggtgtccggccagggcgactctctgcacgagcatatcgctaacctggccggcagccccgctatcaagaagggcatcctgcagacagtgaaggtggtggacgagctcgtgaaagtgatgggcagacacaagcccgagaacatcgtgatcgagatggctagagagaaccagaccacccagaagggacagaagaactcccgcgagaggatgaagagaatcgaagagggcatcaaagagctgggcagccagatcctgaaagaacaccccgtggaaaacacccagctgcagaacgagaagctgtacctgtactacctgcagaatggccgggatatgtacgtggaccaggaactggacatcaacagactgtccgactacgatgtggaccatatcgtgcctcagagctttctgaaggacgactccatcgataacaaagtgctgactcggagcgacaagaacagaggcaagagcgacaacgtgccctccgaagaggtcgtgaagaagatgaagaactactggcgacagctgctgaacgccaagctgattacccagaggaagttcgataacctgaccaaggccgagagaggcggcctgagcgagctggataaggccggcttcatcaagaggcagctggtggaaaccagacagatcacaaagcacgtggcacagatcctggactcccggatgaacactaagtacgacgaaaacgataagctgatccgggaagtgaaagtgatcaccctgaagtccaagctggtgtccgatttccggaaggatttccagttttacaaagtgcgcgagatcaacaactaccaccacgcccacgacgcctacctgaacgccgtcgtgggaaccgccctgatcaaaaagtaccctaagctggaaagcgagttcgtgtacggcgactacaaggtgtacgacgtgcggaagatgatcgccaagagcgagcaggaaatcggcaaggctaccgccaagtacttcttctacagcaacatcatgaactttttcaagaccgaaatcaccctggccaacggcgagatcagaaagcgccctctgatcgagacaaacggcgaaaccggggagatcgtgtgggataagggcagagacttcgccacagtgcgaaaggtgctgagcatgccccaagtgaatatcgtgaaaaagaccgaggtgcagacaggcggcttcagcaaagagtctatcctgcccaagaggaacagcgacaagctgatcgccagaaagaaggactgggaccccaagaagtacggcggcttcgacagccctaccgtggcctactctgtgctggtggtggctaaggtggaaaagggcaagtccaagaaactgaagagtgtgaaagagctgctggggatcaccatcatggaaagaagcagctttgagaagaaccctatcgactttctggaagccaagggctacaaagaagtgaaaaaggacctgatcatcaagctgcctaagtactccctgttcgagctggaaaacggcagaaagagaatgctggcctctgccggcgaactgcagaagggaaacgagctggccctgcctagcaaatatgtgaacttcctgtacctggcctcccactatgagaagctgaagggcagccctgaggacaacgaacagaaacagctgtttgtggaacagcataagcactacctggacgagatcatcgagcagatcagcgagttctccaagagagtgatcctggccgacgccaatctggacaaggtgctgtctgcctacaacaagcacagggacaagcctatcagagagcaggccgagaatatcatccacctgttcaccctgacaaacctgggcgctcctgccgccttcaagtactttgacaccaccatcgaccggaagaggtacaccagcaccaaagaggtgctggacgccaccctgatccaccagagcatcaccggcctgtacgagacaagaatcgacctgtctcagctgggaggcgacaagagacctgccgccactaagaaggccggacaggccaaaaagaagaag

SEQ ID NO: 31 - DNA, 4239 bp, Artificial Sequence
  Synthetic
  misc_feature (1)..(66): 3xFLAG
  misc_feature (67)..(4239): Cas9
gactataaggaccacgacggagactacaaggatcatgatattgattacaaagacgatgacgataagatggacaagcccaagaaaaagcggaaagtgaagtacagcatcggcctggacatcggcaccaactctgtgggctgggccgtgatcaccgacgagtacaaggtgcccagcaagaaattcaaggtgctgggcaacaccgacaggcacagcatcaagaagaacctgatcggcgccctgctgttcgacagcggcgaaacagccgaggccaccagactgaagagaaccgccagaagaagatacaccaggcggaagaacaggatctgctatctgcaagagatcttcagcaacgagatggccaaggtggacgacagcttcttccacagactggaagagtccttcctggtggaagaggacaagaagcacgagagacaccccatcttcggcaacatcgtggacgaggtggcctaccacgagaagtaccccaccatctaccacctgagaaagaaactggtggacagcaccgacaaggccgacctgagactgatctacctggccctggcccacatgatcaagttcagaggccacttcctgatcgagggcgacctgaaccccgacaacagcgacgtggacaagctgttcatccagctggtgcagacctacaaccagctgttcgaggaaaaccccatcaacgccagcggcgtggacgccaaggctatcctgtctgccagactgagcaagagcagaaggctggaaaatctgatcgcccagctgcccggcgagaagaagaacggcctgttcggcaacctgattgccctgagcctgggcctgacccccaacttcaagagcaacttcgacctggccgaggatgccaaactgcagctgagcaaggacacctacgacgacgacctggacaacctgctggcccagatcggcgaccagtacgccgacctgttcctggccgccaagaacctgtctgacgccatcctgctgagcgacatcctgagagtgaacaccgagatcaccaaggcccccctgagcgcctctatgatcaagagatacgacgagcaccaccaggacctgaccctgctgaaagctctcgtgcggcagcagctgcctgagaagtacaaagaaatcttcttcgaccagagcaagaacggctacgccggctacatcgatggcggcgctagccaggaagagttctacaagttcatcaagcccatcctggaaaagatggacggcaccgaggaactgctcgtgaagctgaacagagaggacctgctgagaaagcagagaaccttcgacaacggcagcatcccccaccagatccacctgggagagctgcacgctatcctgagaaggcaggaagatttttacccattcctgaaggacaaccgggaaaagatcgagaagatcctgaccttcaggatcccctactacgtgggccccctggccagaggcaacagcagattcgcctggatgaccagaaagagcgaggaaaccatcaccccctggaacttcgaggaagtggtggacaagggcgccagcgcccagagcttcatcgagagaatgacaaacttcgataagaacctgcccaacgagaaggtgctgcccaagcacagcctgctgtacgagtacttcaccgtgtacaacgagctgaccaaagtgaaatacgtgaccgagggaatgagaaagcccgccttcctgagcggcgagcagaaaaaggccatcgtggacctgctgttcaagaccaacagaaaagtgaccgtgaagcagctgaaagaggactacttcaagaaaatcgagtgcttcgactccgtggaaatctccggcgtggaagatagattcaacgcctccctgggcacataccacgatctgctgaaaattatcaaggacaaggacttcctggataacgaagagaacgaggacattctggaagatatcgtgctgaccctgacactgtttgaggaccgcgagatgatcgaggaaaggctgaaaacctacgctcacctgttcgacgacaaagtgatgaagcagctgaagagaaggcggtacaccggctggggcaggctgagcagaaagctgatcaacggcatcagagacaagcagagcggcaagacaatcctggatttcctgaagtccgacggcttcgccaaccggaacttcatgcagctgatccacgacgacagcctgacattcaaagaggacatccagaaagcccaggtgtccggccagggcgactctctgcacgagcatatcgctaacctggccggcagccccgctatcaagaagggcatcctgcagacagtgaaggtggtggacgagctcgtgaaagtgatgggcagacacaagcccgagaacatcgtgatcgagatggctagagagaaccagaccacccagaagggacagaagaactcccgcgagaggatgaagagaatcgaagagggcatcaaagagctgggcagccagatcctgaaagaacaccccgtggaaaacacccagctgcagaacgagaagctgtacctgtactacctgcagaatggccgggatatgtacgtggaccaggaactggacatcaacagactgtccgactacgatgtggaccatatcgtgcctcagagctttctgaaggacgactccatcgataacaaagtgctgactcggagcgacaagaacagaggcaagagcgacaacgtgccctccgaagaggtcgtgaagaagatgaagaactactggcgacagctgctgaacgccaagctgattacccagaggaagttcgataacctgaccaaggccgagagaggcggcctgagcgagctggataaggccggcttcatcaagaggcagctggtggaaaccagacagatcacaaagcacgtggcacagatcctggactcccggatgaacactaagtacgacgaaaacgataagctgatccgggaagtgaaagtgatcaccctgaagtccaagctggtgtccgatttccggaaggatttccagttttacaaagtgcgcgagatcaacaactaccaccacgcccacgacgcctacctgaacgccgtcgtgggaaccgccctgatcaaaaagtaccctaagctggaaagcgagttcgtgtacggcgactacaaggtgtacgacgtgcggaagatgatcgccaagagcgagcaggaaatcggcaaggctaccgccaagtacttcttctacagcaacatcatgaactttttcaagaccgaaatcaccctggccaacggcgagatcagaaagcgccctctgatcgagacaaacggcgaaaccggggagatcgtgtgggataagggcagagacttcgccacagtgcgaaaggtgctgagcatgccccaagtgaatatcgtgaaaaagaccgaggtgcagacaggcggcttcagcaaagagtctatcctgcccaagaggaacagcgacaagctgatcgccagaaagaaggactgggaccccaagaagtacggcggcttcgacagccctaccgtggcctactctgtgctggtggtggctaaggtggaaaagggcaagtccaagaaactgaagagtgtgaaagagctgctggggatcaccatcatggaaagaagcagctttgagaagaaccctatcgactttctggaagccaagggctacaaagaagtgaaaaaggacctgatcatcaagctgcctaagtactccctgttcgagctggaaaacggcagaaagagaatgctggcctctgccggcgaactgcagaagggaaacgagctggccctgcctagcaaatatgtgaacttcctgtacctggcctcccactatgagaagctgaagggcagccctgaggacaacgaacagaaacagctgtttgtggaacagcataagcactacctggacgagatcatcgagcagatcagcgagttctccaagagagtgatcctggccgacgccaatctggacaaggtgctgtctgcctacaacaagcacagggacaagcctatcagagagcaggccgagaatatcatccacctgttcaccctgacaaacctgggcgctcctgccgccttcaagtactttgacaccaccatcgaccggaagaggtacaccagcaccaaagaggtgctggacgccaccctgatccaccagagcatcaccggcctgtacgagacaagaatcgacctgtctcagctgggaggcgacaagagacctgccgccactaagaaggccggacaggccaaaaagaagaag

SEQ ID NO: 32 - DNA, 66 bp, Artificial Sequence
  Synthetic
ggaagcggagccactaacttctccctgttgaaacaagcaggggatgtcgaagagaatcccgggcca

SEQ ID NO: 33 - DNA, 714 bp, Artificial Sequence
  Synthetic
gtgagcaagggcgaggagctgttcaccggggtggtgcccatcctggtcgagctggacggcgacgtaaacggccacaagttcagcgtgtccggcgagggcgagggcgatgccacctacggcaagctgaccctgaagttcatctgcaccaccggcaagctgcccgtgccctggcccaccctcgtgaccaccctgacctacggcgtgcagtgcttcagccgctaccccgaccacatgaagcagcacgacttcttcaagtccgccatgcccgaaggctacgtccaggagcgcaccatcttcttcaaggacgacggcaactacaagacccgcgccgaggtgaagttcgagggcgacaccctggtgaaccgcatcgagctgaagggcatcgacttcaaggaggacggcaacatcctggggcacaagctggagtacaactacaacagccacaacgtctatatcatggccgacaagcagaagaacggcatcaaggtgaacttcaagatccgccacaacatcgaggacggcagcgtgcagctcgccgaccactaccagcagaacacccccatcggcgacggccccgtgctgctgcccgacaaccactacctgagcacccagtccgccctgagcaaagaccccaacgagaagcgcgatcacatggtcctgctggagttcgtgaccgccgccgggatcactctcggcatggacgagctgtacaag

SEQ ID NO: 34 - DNA, 66 bp, Artificial Sequence
  Synthetic
gactataaggaccacgacggagactacaaggatcatgatattgattacaaagacgatgacgataag

SEQ ID NO: 35 - DNA, 597 bp, Artificial Sequence
  Synthetic
cgataatcaacctctggattacaaaatttgtgaaagattgactggtattcttaactatgttgctccttttacgctatgtggatacgctgctttaatgcctttgtatcatgctattgcttcccgtatggctttcattttctcctccttgtataaatcctggttgctgtctctttatgaggagttgtggcccgttgtcaggcaacgtggcgtggtgtgcactgtgtttgctgacgcaacccccactggttggggcattgccaccacctgtcagctcctttccgggactttcgctttccccctccctattgccacggcggaactcatcgccgcctgccttgcccgctgctggacaggggctcggctgttgggcactgacaattccgtggtgttgtcggggaaatcatcgtcctttccttggctgctcgcctgtgttgccacctggattctgcgcgggacgtccttctgctacgtcccttcggccctcaatccagcggaccttccttcccgcggcctgctgccggctctgcggcctcttccgcgtcttcgccttcgccctcagacgagtcggatctccctttgggccgcctccccgcatcg

SEQ ID NO: 36 - DNA, 216 bp, Artificial Sequence
  Synthetic
cgacctcgacctcgactgtgccttctagttgccagccatctgttgtttgcccctcccccgtgccttccttgaccctggaaggtgccactcccactgtcctttcctaataaaatgaggaaattgcatcgcattgtctgagtaggtgtcattctattctggggggtggggtggggcaggacagcaagggggaggattgggaagacaatggcaggcatg

SEQ ID NO: 37 - DNA, 2066 bp, Artificial Sequence
  Synthetic
atgggatcggccattgaacaagatggattgcacgcaggttctccggccgcttgggtggagaggctattcggctatgactgggcacaacagacaatcggctgctctgatgccgccgtgttccggctgtcagcgcaggggcgcccggttctttttgtcaagaccgacctgtccggtgccctgaatgaactgcaggacgaggcagcgcggctatcgtggctggccacgacgggcgttccttgcgcagctgtgctcgacgttgtcactgaagcgggaagggactggctgctattgggcgaagtgccggggcaggatctcctgtcatctcaccttgctcctgccgagaaagtatccatcatggctgatgcaatgcggcggctgcatacgcttgatccggctacctgcccattcgaccaccaagcgaaacatcgcatcgagcgagcacgtactcggatggaagccggtcttgtcgatcaggatgatctggacgaagagcatcaggggctcgcgccagccgaactgttcgccaggctcaaggcgcgcatgcccgacggcgatgatctcgtcgtgacccatggcgatgcctgcttgccgaatatcatggtggaaaatggccgcttttctggattcatcgactgtggccggctgggtgtggcggaccgctatcaggacatagcgttggctacccgtgatattgctgaagagcttggcggcgaatgggctgaccgcttcctcgtgctttacggtatcgccgctcccgattcgcagcgcatcgccttctatcgccttcttgacgagttcttctgaggggatccgctgtaagtctgcagaaattgatgatctattaaacaataaagatgtccactaaaatggaagtttttcctgtcatactttgttaagaagggtgagaacagagtacctacattttgaatggaaggattggagctacgggggtgggggtggggtgggattagataaatgcctgctctttactgaaggctctttactattgctttatgataatgtttcatagttggatatcataatttaaacaagcaaaaccaaattaagggccagctcattcctcccactcatgatctatagatctatagatctctcgtgggatcattgtttttctcttgattcccactttgtggttctaagtactgtggtttccaaatgtgtcagtttcatagcctgaagaacgagatcagcagcctctgttccacatacacttcattctcagtattgttttgccaagttctaattccatcagaagcttgcagatctgcgactctagaggatctgcgactctagaggatcataatcagccataccacatttgtagaggttttacttgctttaaaaaacctcccacacctccccctgaacctgaaacataaaatgaatgcaattgttgttgttaacttgtttattgcagcttataatggttacaaataaagcaatagcatcacaaatttcacaaataaagcatttttttcactgcattctagttgtggtttgtccaaactcatcaatgtatcttatcatgtctggatctgcgactctagaggatcataatcagccataccacatttgtagaggttttacttgctttaaaaaacctcccacacctccccctgaacctgaaacataaaatgaatgcaattgttgttgttaacttgtttattgcagcttataatggttacaaataaagcaatagcatcacaaatttcacaaataaagcatttttttcactgcattctagttgtggtttgtccaaactcatcaatgtatcttatcatgtctggatctgcgactctagaggatcataatcagccataccacatttgtagaggttttacttgctttaaaaaacctcccacacctccccctgaacctgaaacataaaatgaatgcaattgttgttgttaacttgtttattgcagcttataatggttacaaataaagcaatagcatcacaaatttcacaaataaagcatttttttcactgcattctagttgtggtttgtccaaactcatcaatgtatcttatcatgtctggatcc

SEQ ID NO: 38 - DNA, 1719 bp, Artificial Sequence
  Synthetic
actagttattaatagtaatcaattacggggtcattagttcatagcccatatatggagttccgcgttacataacttacggtaaatggcccgcctggctgaccgcccaacgacccccgcccattgacgtcaataatgacgtatgttcccatagtaacgccaatagggactttccattgacgtcaatgggtggagtatttacggtaaactgcccacttggcagtacatcaagtgtatcatatgccaagtacgccccctattgacgtcaatgacggtaaatggcccgcctggcattatgcccagtacatgaccttatgggactttcctacttggcagtacatctacgtattagtcatcgctattaccatggtcgaggtgagccccacgttctgcttcactctccccatctcccccccctccccacccccaattttgtatttatttattttttaattattttgtgcagcgatgggggcggggggggggggggggcgcgcgccaggcggggcggggcggggcgaggggcggggcggggcgaggcggagaggtgcggcggcagccaatcagagcggcgcgctccgaaagtttccttttatggcgaggcggcggcggcggcggccctataaaaagcgaagcgcgcggcgggcggggagtcgctgcgacgctgccttcgccccgtgccccgctccgccgccgcctcgcgccgcccgccccggctctgactgaccgcgttactcccacaggtgagcgggcgggacggcccttctcctccgggctgtaattagcgcttggtttaatgacggcttgtttcttttctgtggctgcgtgaaagccttgaggggctccgggagggccctttgtgcggggggagcggctcggggggtgcgtgcgtgtgtgtgtgcgtggggagcgccgcgtgcggctccgcgctgcccggcggctgtgagcgctgcgggcgcggcgcggggctttgtgcgctccgcagtgtgcgcgaggggagcgcggccgggggcggtgccccgcggtgcggggggggctgcgaggggaacaaaggctgcgtgcggggtgtgtgcgtgggggggtgagcagggggtgtgggcgcgtcggtcgggctgcaaccccccctgcacccccctccccgagttgctgagcacggcccggcttcgggtgcggggctccgtacggggcgtggcgcggggctcgccgtgccgggcggggggtggcggcaggtgggggtgccgggcggggcggggccgcctcgggccggggagggctcgggggaggggcgcggcggcccccggagcgccggcggctgtcgaggcgcggcgagccgcagccattgccttttatggtaatcgtgcgagagggcgcagggacttcctttgtcccaaatctgtgcggagccgaaatctgggaggcgccgccgcaccccctctagcgggcgcggggcgaagcggtgcggcgccggcaggaaggaaatgggcggggagggccttcgtgcgtcgccgcgccgccgtccccttctccctctccagcctcggggctgtccgcggggggacggctgccttcgggggggacggggcagggcggggttcggcttctggcgtgtgaccggcggctctagagcctctgctaaccatgttcatgccttcttctttttcctacagctcctgggcaacgtgctggttattgtgctgtctcatcattttggcaaagaattcg